European Patent Specification EP 3 247 388 B1, published September 10, 2025. Title: RECOMBINANT PARAMYXOVIRUSES AND THEIR USE. Applicant: The United States of America, as represented by the Secretary, Department of Health and Human Services Collins, Peter Liang, Bo Munir, Shirin Schaap-Nutt, Anne Buchholz, Ursula Mackow, Natalie Kwong, Peter McLellan, Jason Graham, Barney. The sequence listing filed with the application follows.

SEQUENCE LISTING (150 sequences)

SEQ ID NO: 1 - protein, 574 aa, Artificial sequence
  Recombinant RSV F
MELLILKANAITTILTAVTFCFASGQNITEEFYQSTCSAVSKGYLSALRTGWYTSVITIELSNIKENKCNGTDAKVKLIKQELDKYKNAVTELQLLMQSTPATNNRARRELPRFMNYTLNNAKKTNVTLSKKRKRRFLGFLLGVGSAIASGVAVSKVLHLEGEVNKIKSALLSTNKAVVSLSNGVSVLTSKVLDLKNYIDKQLLPIVNKQSCSISNIETVIEFQQKNNRLLEITREFSVNAGVTTPVSTYMLTNSELLSLINDMPITNDQKKLMSNNVQIVRQQSYSIMSIIKEEVLAYVVQLPLYGVIDTPCWKLHTSPLCTTNTKEGSNICLTRTDRGWYCDNAGSVSFFPQAETCKVQSNRVFCDTMNSLTLPSEVNLCNVDIFNPKYDCKIMTSKTDVSSSVITSLGAIVSCYGKTKCTASNKNRGIIKTFSNGCDYVSNKGVDTVSVGNTLYYVNKQEGKSLYVKGEPIINFYDPLVFPSDEFDASISQVNEKINQSLAFIRKSDELLHNVNAGKSTTNIMITTIIIVIIVILLSLIAVGLLLYCKARSTPVTLSKDQLSGINNIAFSN

SEQ ID NO: 2 - protein, 574 aa, Respiratory syncytial virus
MELLIHRLSAIFLTLAINALYLTSSQNITEEFYQSTCSAVSRGYFSALRTGWYTSVITIELSNIKETKCNGTDTKVKLIKQELDKYKNAVTELQLLMQNTPAANNRARREAPQYMNYTINTTKNLNVSISKKRKRRFLGFLLGVGSAIASGIAVSKVLHLEGEVNKIKNALLSTNKAVVSLSNGVSVLTSKVLDLKNYINNQLLPIVNQQSCRISNIETVIEFQQKNSRLLEINREFSVNAGVTTPLSTYMLTNSELLSLINDMPITNDQKKLMSSNVQIVRQQSYSIMSIIKEEVLAYVVQLPIYGVIDTPCWKLHTSPLCTTNIKEGSNICLTRTDRGWYCDNAGSVSFFPQADTCKVQSNRVFCDTMNSLTLPSEVSLCNTDIFNSKYDCKIMTSKTDISSSVITSLGAIVSCYGKTKCTASNKNRGIIKTFSNGCDYVSNKGVDTVSVGNTLYYVNKLEGKNLYVKGEPIINYYDPLVFPSDEFDASISQVNEKINQSLAFIRRSDELLHNVNTGKSTTNIMITTIIIVIIVVLLSLIAIGLLLYCKAKNTPVTLSKDQLSGINNIAFSK

SEQ ID NO: 3 - RNA, 1725 nt, Respiratory syncytial virus
auggagcugcugauccacagguuaagugcaaucuuccuaacucuugcuauuaaugcauuguaccucaccucaagucagaacauaacugaggaguuuuaccaaucgacauguagugcaguuagcagagguuauuuuagugcuuuaagaacagguugguauaccagugucauaacaauagaauuaaguaauauaaaagaaaccaaaugcaauggaacugacacuaaaguaaaacuuauaaaacaagaauuagauaaguauaagaaugcagugacagaauuacagcuacuuaugcaaaacacaccagcugccaacaaccgggccagaagagaagcaccacaguauaugaacuauacaaucaauaccacuaaaaaccuaaauguaucaauaagcaagaagaggaaacgaagauuucugggcuucuuguuagguguaggaucugcaauagcaagugguauagcuguauccaaaguucuacaccuugaaggagaagugaacaagaucaaaaaugcuuuguuaucuacaaacaaagcuguagucagucuaucaaauggggucaguguuuuaaccagcaaaguguuagaucucaagaauuacauaaauaaccaauuauuacccauaguaaaucaacagagcugucgcaucuccaacauugaaacaguuauagaauuccagcagaagaacagcagauuguuggaaaucaacagagaauucagugucaaugcagguguaacaacaccuuuaagcacuuacauguuaacaaacagugaguuacuaucauugaucaaugauaugccuauaacaaaugaucagaaaaaauuaaugucaagcaauguucagauaguaaggcaacaaaguuauucuaucaugucuauaauaaaggaagaaguccuugcauauguuguacagcuaccuaucuaugguguaauagauacaccuugcuggaaauuacacacaucaccucuaugcaccaccaacaucaaagaaggaucaaauauuuguuuaacaaggacugauagaggaugguauugugauaaugcaggaucaguauccuucuuuccacaggcugacacuuguaaaguacaguccaaucgaguauuuugugacacuaugaacaguuugacauuaccaagugaagucagccuuuguaacacugacauauucaauuccaaguaugacugcaaaauuaugacaucaaaaacagacauaagcagcucaguaauuacuucucuuggagcuauagugucaugcuaugguaaaacuaaaugcacugcauccaacaaaaaucgugggauuauaaagacauuuucuaaugguugugacuaugugucaaacaaaggaguagauacugugucagugggcaacacuuuauacuauguaaacaagcuggaaggcaagaaccuuuauguaaaaggggaaccuauaauaaauuacuaugacccucuaguguuuccuucugaugaguuugaugcaucaauaucucaagucaaugaaaaaaucaaucaaaguuuagcuuuuauucguagaucugaugaauuacuacauaauguaaauacuggcaaaucuacuacaaauauuaugauaacuacaauuauuauaguaaucauuguaguauuguuaucauuaauagcuauugguuugcuguuguauugcaaagccaaaaacacaccaguuacacuaagcaaagaccaacuaaguggaaucaauaauauugcauucagcaaauag

SEQ ID NO: 4 - DNA, 1725 bp, Artificial sequence
  Recombinant RSV F
atggaactgctgatcctgaaggccaacgccatcacaacaatcctgaccgccgtgaccttctgcttcgccagcggccagaacatcaccgaggaattctaccagagcacctgtagcgccgtgtccaagggctacctgagcgccctgagaaccggctggtacaccagcgtgatcaccatcgagctgtccaacatcaaagaaaacaagtgcaacggcaccgacgccaaagtgaagctgatcaagcaggaactggacaagtacaagaacgccgtgaccgagctgcagctgctgatgcagtccacccccgccaccaacaaccgggccagaagagaactgccccggttcatgaactacaccctcaacaacgccaaaaagaccaacgtgaccctgagcaagaagcggaagcggcggttcctgggcttcctgctgggcgtgggcagcgccattgcctctggcgtggccgtgtctaaggtgctgcacctggaaggcgaagtgaacaagatcaagagcgccctgctgtccacaaacaaggccgtggtgtccctgagcaacggcgtgtccgtgctgacctccaaggtgctggatctgaagaactacatcgacaagcagctgctgcccatcgtgaacaagcagagctgcagcatcagcaacatcgagacagtgatcgagttccagcagaagaacaaccggctgctggaaatcacccgcgagttcagcgtgaacgccggcgtgaccacccccgtgtccacctacatgctgaccaacagcgagctgctgtccctgatcaatgacatgcccatcaccaacgaccagaaaaagctgatgagcaacaacgtgcagatcgtgcggcagcagagctactccatcatgagcatcatcaaagaagaggtgctggcctacgtggtgcagctgcccctgtacggcgtgatcgacaccccctgctggaagctgcacaccagccccctgtgcaccaccaacacaaaagagggcagcaacatctgcctgacccggaccgaccggggctggtactgcgataatgccggcagcgtgtcattctttccacaggccgagacatgcaaggtgcagagcaaccgggtgttctgcgacaccatgaacagcctgaccctgccctccgaagtgaacctgtgcaacgtggacatcttcaaccctaagtacgactgcaagatcatgaccagcaagaccgacgtgtccagctccgtgatcacctccctgggcgccatcgtgtcctgctacggcaagaccaagtgcaccgccagcaacaagaaccggggcatcatcaagaccttcagcaacggctgcgactacgtgtccaacaagggggtggacaccgtgtccgtgggcaacaccctgtactacgtgaacaaacaggaaggcaagagcctgtacgtgaagggcgagcccatcatcaacttctacgaccccctggtgttccccagcgacgagttcgacgccagcatcagccaggtcaacgagaagatcaaccagagcctggccttcatcagaaagagcgacgagctgctgcacaatgtgaatgccggcaagagcaccacaaacatcatgatcaccactatcatcatcgtgatcatcgtcatcctgctgagtctgatcgccgtgggcctgctgctgtactgcaaggccagatccacccctgtgaccctgtccaaggatcagctgtccggcatcaacaatatcgccttctccaactga

SEQ ID NO: 5 - DNA, 1725 bp, Artificial sequence
  Recombinant RSV F
atggaactgctgatcctgaaagccaacgctattactactatcctgaccgccgtgacattttgcttcgcatctggacagaacattactgaggaattctaccagtcaacatgcagcgccgtgtccaaaggatacctgagcgccctgcggaccggctggtatacatcagtgattactatcgagctgtccaacatcaaggaaaacaaatgtaatgggaccgacgcaaaggtgaaactgatcaagcaggagctggataagtacaaaaatgccgtgacagaactgcagctgctgatgcagtccacaccagcaactaacaatcgcgcccggagagagctgccccggttcatgaactataccctgaacaatgctaagaaaaccaatgtgacactgtccaagaaacgcaagaggcgcttcctgggatttctgctgggcgtggggtctgccatcgctagtggagtggccgtctctaaagtcctgcacctggagggcgaagtgaacaagatcaaaagcgccctgctgtccactaacaaggcagtggtcagtctgtcaaatggcgtgtccgtcctgacctctaaggtgctggacctgaaaaattatattgataagcagctgctgcctatcgtcaacaaacagagctgctccatttctaatatcgagacagtgatcgaattccagcagaagaacaatagactgctggagattaccagagagttcagcgtgaacgccggcgtcaccacacccgtgtccacctacatgctgacaaatagtgagctgctgtcactgattaacgacatgcctatcaccaatgatcagaagaaactgatgtccaacaatgtgcagatcgtcagacagcagagttactcaatcatgtctatcattaaggaggaagtcctggcctacgtggtccagctgccactgtatggcgtgatcgacaccccctgctggaaactgcatacatctcctctgtgcactaccaacacaaaggaaggaagtaatatctgcctgactcgaaccgaccggggatggtactgtgataacgcaggcagcgtgtccttctttccacaggccgagacctgcaaggtccagagcaacagggtgttctgtgacactatgaatagcctgaccctgccttccgaagtcaacctgtgcaatgtggacatctttaatccaaagtacgattgtaagatcatgactagcaagaccgatgtcagctcctctgtgattacttctctgggggccatcgtgagttgctacggaaagacaaaatgtactgccagcaacaaaaatcgcggcatcattaagaccttctccaacgggtgcgactatgtctctaacaagggcgtggatacagtgagtgtcgggaacactctgtactatgtcaataagcaggagggaaaaagcctgtacgtgaagggcgaacccatcattaacttctatgaccccctggtgttcccttccgacgagtttgatgcatctattagtcaggtgaacgaaaaaatcaatcagagtctggcctttattcggaagtcagatgagctgctgcacaacgtgaatgctggcaaatctacaactaacatcatgatcaccacaatcatcatcgtgattatcgtcattctgctgtcactgatcgctgtggggctgctgctgtactgtaaggcaagaagcaccccagtcactctgtcaaaagaccagctgtcagggattaacaacattgccttcagtaactga

SEQ ID NO: 6 - DNA, 1725 bp, Artificial sequence; identical to SEQ ID NO: 4
  Recombinant RSV F

SEQ ID NO: 7 - DNA, 1725 bp, Artificial sequence; identical to SEQ ID NO: 5
  Recombinant RSV F

SEQ ID NO: 8 - protein, 573 aa, Artificial sequence
  Recombinant RSV F
MELLILKANAITTILTAVTFCFASGQNITEEFYQSTCSAVSKGYLSALRTGWYTSVITIELSNIKENKCNGTDAKVKLIKQELDKYKNAVTELQLLMQSTPATNNRARRELPRFMNYTLNNAKKTNVTLSKKRKRRFLGFLLGVGSAIASGVAVCKVLHLEGEVNKIKSALLSTNKAVVSLSNGVSVLTFKVLDLKNYIDKQLLPILNKQSCSISNIETVIEFQQKNNRLLEITREFSVNAGVTTPVSTYMLTNSELLSLINDMPITNDQKKLMSNNVQIVRQQSYSIMCIIKEEVLAYVVQLPLYGVIDTPCWKLHTSPLCTTNTKEGSNICLTRTDRGWYCDNAGSVSFFPQAETCKVQSNRVFCDTMNSLTLPSEVNLCNVDIFNPKYDCKIMTSKTDVSSSVITSLGAIVSCYGKTKCTASNKNRGIIKTFSNGCDYVSNKGVDTVSVGNTLYYVNKQEGKSLYVKGEPIINFYDPLVFPSDEFDASISQVNEKINQSLAFIRKSDELLHNVNAGKSTTNIMITTIIIVIIVILLSLIAVGLLLYCKYYRIQKRNRVDQNDKPYVLTNK

SEQ ID NO: 9 - DNA, 1722 bp, Artificial sequence
  Recombinant RSV F
atggaactgctgatcctgaaagccaacgctattactactatcctgaccgccgtgacattttgcttcgcatctggacagaacattactgaggaattctaccagtcaacatgcagcgccgtgtccaaaggatacctgagcgccctgcggaccggctggtatacatcagtgattactatcgagctgtccaacatcaaggaaaacaaatgtaatgggaccgacgcaaaggtgaaactgatcaagcaggagctggataagtacaaaaatgccgtgacagaactgcagctgctgatgcagtccacaccagcaactaacaatcgcgcccggagagagctgccccggttcatgaactataccctgaacaatgctaagaaaaccaatgtgacactgtccaagaaacgcaagaggcgcttcctgggatttctgctgggcgtggggtctgccatcgctagtggagtggccgtctgcaaagtcctgcacctggagggcgaagtgaacaagatcaaaagcgccctgctgtccactaacaaggcagtggtcagtctgtcaaatggcgtgtccgtcctgaccttcaaggtgctggacctgaaaaattatattgataagcagctgctgcctatcctgaacaaacagagctgctccatttctaatatcgagacagtgatcgaattccagcagaagaacaatagactgctggagattaccagagagttcagcgtgaacgccggcgtcaccacacccgtgtccacctacatgctgacaaatagtgagctgctgtcactgattaacgacatgcctatcaccaatgatcagaagaaactgatgtccaacaatgtgcagatcgtcagacagcagagttactcaatcatgtgcatcattaaggaggaagtcctggcctacgtggtccagctgccactgtatggcgtgatcgacaccccctgctggaaactgcatacatctcctctgtgcactaccaacacaaaggaaggaagtaatatctgcctgactcgaaccgaccggggatggtactgtgataacgcaggcagcgtgtccttctttccacaggccgagacctgcaaggtccagagcaacagggtgttctgtgacactatgaatagcctgaccctgccttccgaagtcaacctgtgcaatgtggacatctttaatccaaagtacgattgtaagatcatgactagcaagaccgatgtcagctcctctgtgattacttctctgggggccatcgtgagttgctacggaaagacaaaatgtactgccagcaacaaaaatcgcggcatcattaagaccttctccaacgggtgcgactatgtctctaacaagggcgtggatacagtgagtgtcgggaacactctgtactatgtcaataagcaggagggaaaaagcctgtacgtgaagggcgaacccatcattaacttctatgaccccctggtgttcccttccgacgagtttgatgcatctattagtcaggtgaacgaaaaaatcaatcagagtctggcctttattcggaagtcagatgagctgctgcacaacgtgaatgctggcaaatctacaactaacatcatgatcaccacaatcatcatcgtgattatcgtcattctgctgtcactgatcgctgtggggctgctgctgtactgtaagtactaccgtatccagaagaggaacagagttgaccagaacgataagccatacgtgctcactaacaagtga

SEQ ID NO: 10 - protein, 575 aa, Artificial sequence
  Recombinant RSV F
MELLILKANAITTILTAVTFCFASGQNITEEFYQSTCSAVSKGYLSALRTGWYTSVITIELSNIKENKCNGTDAKVKLIKQELDKYKNAVTELQLLMQSTPATNNRARRELPRFMNYTLNNAKKTNVTLSKKRKRRFLGFLLGVGSAIASGVAVCKVLHLEGEVNKIKSALLSTNKAVVSLSNGVSVLTFKVLDLKNYIDKQLLPILNKQSCSISNIETVIEFQQKNNRLLEITREFSVNAGVTTPVSTYMLTNSELLSLINDMPITNDQKKLMSNNVQIVRQQSYSIMCIIKEEVLAYVVQLPLYGVIDTPCWKLHTSPLCTTNTKEGSNICLTRTDRGWYCDNAGSVSFFPQAETCKVQSNRVFCDTMNSLTLPSEVNLCNVDIFNPKYDCKIMTSKTDVSSSVITSLGAIVSCYGKTKCTASNKNRGIIKTFSNGCDYVSNKGVDTVSVGNTLYYVNKQEGKSLYVKGEPIINFYDPLVFPSDEFDASISQVNEKINQSLAFIRKSDELLHNVNAGKSTTNIMITTIIIILIMIIILFIINITIITIAIKYYRIQKRNRVDQNDKPYVLTNK

SEQ ID NO: 11 - DNA, 1728 bp, Artificial sequence
  Recombinant RSV F
atggaactgctgatcctgaaagccaacgctattactactatcctgaccgccgtgacattttgcttcgcatctggacagaacattactgaggaattctaccagtcaacatgcagcgccgtgtccaaaggatacctgagcgccctgcggaccggctggtatacatcagtgattactatcgagctgtccaacatcaaggaaaacaaatgtaatgggaccgacgcaaaggtgaaactgatcaagcaggagctggataagtacaaaaatgccgtgacagaactgcagctgctgatgcagtccacaccagcaactaacaatcgcgcccggagagagctgccccggttcatgaactataccctgaacaatgctaagaaaaccaatgtgacactgtccaagaaacgcaagaggcgcttcctgggatttctgctgggcgtggggtctgccatcgctagtggagtggccgtctgcaaagtcctgcacctggagggcgaagtgaacaagatcaaaagcgccctgctgtccactaacaaggcagtggtcagtctgtcaaatggcgtgtccgtcctgaccttcaaggtgctggacctgaaaaattatattgataagcagctgctgcctatcctgaacaaacagagctgctccatttctaatatcgagacagtgatcgaattccagcagaagaacaatagactgctggagattaccagagagttcagcgtgaacgccggcgtcaccacacccgtgtccacctacatgctgacaaatagtgagctgctgtcactgattaacgacatgcctatcaccaatgatcagaagaaactgatgtccaacaatgtgcagatcgtcagacagcagagttactcaatcatgtgcatcattaaggaggaagtcctggcctacgtggtccagctgccactgtatggcgtgatcgacaccccctgctggaaactgcatacatctcctctgtgcactaccaacacaaaggaaggaagtaatatctgcctgactcgaaccgaccggggatggtactgtgataacgcaggcagcgtgtccttctttccacaggccgagacctgcaaggtccagagcaacagggtgttctgtgacactatgaatagcctgaccctgccttccgaagtcaacctgtgcaatgtggacatctttaatccaaagtacgattgtaagatcatgactagcaagaccgatgtcagctcctctgtgattacttctctgggggccatcgtgagttgctacggaaagacaaaatgtactgccagcaacaaaaatcgcggcatcattaagaccttctccaacgggtgcgactatgtctctaacaagggcgtggatacagtgagtgtcgggaacactctgtactatgtcaataagcaggagggaaaaagcctgtacgtgaagggcgaacccatcattaacttctatgaccccctggtgttcccttccgacgagtttgatgcatctattagtcaggtgaacgaaaaaatcaatcagagtctggcctttattcggaagtcagatgagctgctgcacaacgtgaatgctggcaaatctacaactaacatcatgatcaccacaatcatcatcatcttgatcatgatcatcatcctgttcatcatcaacatcacaatcatcaccatcgctatcaagtactaccgtatccagaagaggaacagagttgaccagaacgataagccatacgtgctcactaacaagtga

SEQ ID NO: 12 - protein, 576 aa, Artificial sequence
  Recombinant RSV F
MELLILKANAITTILTAVTFCFASGQNITEEFYQSTCSAVSKGYLSALRTGWYTSVITIELSNIKENKCNGTDAKVKLIKQELDKYKNAVTELQLLMQSTPATNNRARRELPRFMNYTLNNAKKTNVTLSKKRKRRFLGFLLGVGSAIASGVAVSKVLHLEGEVNKIKSALLSTNKAVVSLSNGVSVLTSKVLDLKNYIDKQLLPIVNKQSCSISNIETVIEFQQKNNRLLEITREFSVNAGVTTPVSTYMLTNSELLSLINDMPITNDQKKLMSNNVQIVRQQSYSIMSIIKEEVLAYVVQLPLYGVIDTPCWKLHTSPLCTTNTKEGSNICLTRTDRGWYCDNAGSVSFFPQAETCKVQSNRVFCDTMNSLTLPSEVNLCNVDIFNPKYDCKIMTSKTDVSSSVITSLGAIVSCYGKTKCTASNKNRGIIKTFSNGCDYVSNKGVDTVSVGNTLYYVNKQEGKSLYVKGEPIINFYDPLVFPSDEFDASISQVNEKINQSLAFIRKSDELLHNVNAGKSTTNIMITTITIIIVMIIILVIINITIIVVIIKFHRIQGKDQNDKNSEPYILTNRQ

SEQ ID NO: 13 - DNA, 1731 bp, Artificial sequence
  Recombinant RSV F
atggaactgctgatcctgaaggccaacgccatcaccaccatcctgaccgccgtgaccttctgctttgccagcggccagaacatcaccgaggaattctaccagagcacctgtagcgccgtgtccaagggctacctgagcgccctgagaaccggctggtacaccagcgtgatcaccatcgagctgagcaacatcaaagaaaacaagtgcaacggcaccgacgccaaagtgaagctgatcaagcaggaactggacaagtacaagaatgccgtgaccgaactgcagctgctgatgcagagcacccccgccaccaacaaccgggccagaagagaactgcccagattcatgaactacaccctgaacaacgccaaaaagaccaacgtgaccctgagcaagaagcggaagcggcggttcctgggctttctgctgggagtgggaagcgccattgctagcggagtggccgtgtctaaggtgctgcacctggaaggcgaagtgaacaagatcaagtccgccctgctgagcaccaacaaggccgtggtgtctctgagcaacggcgtgtccgtgctgaccagcaaggtgctggatctgaagaactacatcgacaaacagctgctgcccatcgtgaacaagcagagctgcagcatcagcaacatcgagacagtgatcgagttccagcagaagaacaaccggctgctggaaatcacccgcgagttcagcgtgaacgctggcgtgaccacccccgtgtccacctacatgctgaccaacagcgagctgctgtccctgatcaacgacatgcccatcaccaacgaccagaaaaagctgatgagcaacaacgtgcagatcgtgcggcagcagagctactccatcatgagcattatcaaagaagaggtgctggcctacgtggtgcagctgcctctgtacggcgtgatcgacaccccctgctggaagctgcacaccagccctctgtgcaccaccaacaccaaagagggctccaacatctgcctgacccggaccgacagaggctggtactgcgataatgccggctccgtctcattctttccacaagccgagacatgcaaggtgcagagcaaccgggtgttctgcgacaccatgaacagcctgaccctgccctccgaagtgaatctgtgcaacgtggacatcttcaaccctaagtacgactgcaagatcatgacctccaagaccgacgtgtccagctccgtgatcacaagcctgggcgccatcgtgtcctgctacggcaagaccaagtgcaccgccagcaacaagaaccggggcatcatcaagaccttcagcaacggctgcgactacgtgtccaacaagggggtggacaccgtgtctgtgggcaacaccctgtactacgtgaacaaacaggaaggcaagagcctgtacgtgaagggcgagcccatcatcaacttctacgaccccctggtgttccccagcgacgagttcgatgccagcatctcccaagtgaacgagaagatcaaccagagcctggccttcatcagaaagtccgatgagctgctgcacaatgtgaacgccggcaagtccaccaccaatatcatgatcaccacaatcaccatcatcattgtgatgattatcatcctcgtgatcatcaacatcacaatcatcgtcgtgattattaagttccaccggatccagggcaaggaccagaacgacaagaactccgagccctacatcctgacaaaccggcagtga

SEQ ID NO: 14 - protein, 576 aa, Artificial sequence
  Recombinant RSV F
MELLILKANAITTILTAVTFCFASGQNITEEFYQSTCSAVSKGYLSALRTGWYTSVITIELSNIKENKCNGTDAKVKLIKQELDKYKNAVTELQLLMQSTPATNNRARRELPRFMNYTLNNAKKTNVTLSKKRKRRFLGFLLGVGSAIASGVAVCKVLHLEGEVNKIKSALLSTNKAVVSLSNGVSVLTSKVLDLKNYIDKQLLPIVNKQSCSISNIETVIEFQQKNNRLLEITREFSVNAGVTTPVSTYMLTNSELLSLINDMPITNDQKKLMSNNVQIVRQQSYSIMCIIKEEVLAYVVQLPLYGVIDTPCWKLHTSPLCTTNTKEGSNICLTRTDRGWYCDNAGSVSFFPQAETCKVQSNRVFCDTMNSLTLPSEVNLCNVDIFNPKYDCKIMTSKTDVSSSVITSLGAIVSCYGKTKCTASNKNRGIIKTFSNGCDYVSNKGVDTVSVGNTLYYVNKQEGKSLYVKGEPIINFYDPLVFPSDEFDASISQVNEKINQSLAFIRKSDELLHNVNAGKSTTNIMITTIIIVIIVILLSLIAVGLLLYCIIKFHRIQGKDQNDKNSEPYILTNRQ

SEQ ID NO: 15 - DNA, 1731 bp, Artificial sequence
  Recombinant RSV F
atggaactgctgatcctgaaggccaacgccatcaccaccatcctgaccgccgtgaccttctgctttgccagcggccagaacatcaccgaggaattctaccagagcacctgtagcgccgtgtccaagggctacctgagcgccctgagaaccggctggtacaccagcgtgatcaccatcgagctgagcaacatcaaagaaaacaagtgcaacggcaccgacgccaaagtgaagctgatcaagcaggaactggacaagtacaagaatgccgtgaccgaactgcagctgctgatgcagagcacccccgccaccaacaaccgggccagaagagaactgcccagattcatgaactacaccctgaacaacgccaaaaagaccaacgtgaccctgagcaagaagcggaagcggcggttcctgggctttctgctgggagtgggaagcgccattgctagcggagtggccgtgtgcaaggtgctgcacctggaaggcgaagtgaacaagatcaagtccgccctgctgagcaccaacaaggccgtggtgtctctgagcaacggcgtgtccgtgctgaccagcaaggtgctggatctgaagaactacatcgacaaacagctgctgcccatcgtgaacaagcagagctgcagcatcagcaacatcgagacagtgatcgagttccagcagaagaacaaccggctgctggaaatcacccgcgagttcagcgtgaacgctggcgtgaccacccccgtgtccacctacatgctgaccaacagcgagctgctgtccctgatcaacgacatgcccatcaccaacgaccagaaaaagctgatgagcaacaacgtgcagatcgtgcggcagcagagctactccatcatgtgcatcatcaaagaagaggtgctggcctacgtggtgcagctgcctctgtacggcgtgatcgacaccccctgctggaagctgcacaccagccctctgtgcaccaccaacaccaaagagggctccaacatctgcctgacccggaccgacagaggctggtactgcgataatgccggctccgtctcattctttccacaagccgagacatgcaaggtgcagagcaaccgggtgttctgcgacaccatgaacagcctgaccctgccctccgaagtgaatctgtgcaacgtggacatcttcaaccctaagtacgactgcaagatcatgacctccaagaccgacgtgtccagctccgtgatcacaagcctgggcgccatcgtgtcctgctacggcaagaccaagtgcaccgccagcaacaagaaccggggcatcatcaagaccttcagcaacggctgcgactacgtgtccaacaagggggtggacaccgtgtctgtgggcaacaccctgtactacgtgaacaaacaggaaggcaagagcctgtacgtgaagggcgagcccatcatcaacttctacgaccccctggtgttccccagcgacgagttcgatgccagcatctcccaagtgaacgagaagatcaaccagagcctggccttcatcagaaagtccgatgagctgctgcacaatgtgaacgccggcaagtccaccaccaatatcatgatcaccacaatcatcatcgtgattatcgtgatcctgctgagcctgatcgccgtgggcctgctgctgtactgtatcatcaagttccaccggatccagggcaaggaccagaacgacaagaactccgagccctacatcctgacaaaccggcagtga

SEQ ID NO: 16 - protein, 576 aa, Artificial sequence
  Recombinant RSV F
MELLILKANAITTILTAVTFCFASGQNITEEFYQSTCSAVSKGYLSALRTGWYTSVITIELSNIKENKCNGTDAKVKLIKQELDKYKNAVTELQLLMQSTPATNNRARRELPRFMNYTLNNAKKTNVTLSKKRKRRFLGFLLGVGSAIASGVAVCKVLHLEGEVNKIKSALLSTNKAVVSLSNGVSVLTFKVLDLKNYIDKQLLPILNKQSCSISNIETVIEFQQKNNRLLEITREFSVNAGVTTPVSTYMLTNSELLSLINDMPITNDQKKLMSNNVQIVRQQSYSIMCIIKEEVLAYVVQLPLYGVIDTPCWKLHTSPLCTTNTKEGSNICLTRTDRGWYCDNAGSVSFFPQAETCKVQSNRVFCDTMNSLTLPSEVNLCNVDIFNPKYDCKIMTSKTDVSSSVITSLGAIVSCYGKTKCTASNKNRGIIKTFSNGCDYVSNKGVDTVSVGNTLYYVNKQEGKSLYVKGEPIINFYDPLVFPSDEFDASISQVNEKINQSLAFIRKSDELLHNVNAGKSTTNIMITTIIIVIIVILLSLIAVGLLLYCIIKFHRIQGKDQNDKNSEPYILTNRQ

SEQ ID NO: 17 - DNA, 1731 bp, Artificial sequence
  Recombinant RSV F
atggaactgctgatcctgaaggccaacgccatcaccaccatcctgaccgccgtgaccttctgctttgccagcggccagaacatcaccgaggaattctaccagagcacctgtagcgccgtgtccaagggctacctgagcgccctgagaaccggctggtacaccagcgtgatcaccatcgagctgagcaacatcaaagaaaacaagtgcaacggcaccgacgccaaagtgaagctgatcaagcaggaactggacaagtacaagaatgccgtgaccgaactgcagctgctgatgcagagcacccccgccaccaacaaccgggccagaagagaactgcccagattcatgaactacaccctgaacaacgccaaaaagaccaacgtgaccctgagcaagaagcggaagcggcggttcctgggctttctgctgggagtgggaagcgccattgctagcggagtggccgtgtgcaaggtgctgcacctggaaggcgaagtgaacaagatcaagtccgccctgctgagcaccaacaaggccgtggtgtctctgagcaacggcgtgtccgtgctgaccttcaaggtgctggatctgaagaactacatcgacaaacagctgctgcccatcttgaacaagcagagctgcagcatcagcaacatcgagacagtgatcgagttccagcagaagaacaaccggctgctggaaatcacccgcgagttcagcgtgaacgctggcgtgaccacccccgtgtccacctacatgctgaccaacagcgagctgctgtccctgatcaacgacatgcccatcaccaacgaccagaaaaagctgatgagcaacaacgtgcagatcgtgcggcagcagagctactccatcatgtgcatcatcaaagaagaggtgctggcctacgtggtgcagctgcctctgtacggcgtgatcgacaccccctgctggaagctgcacaccagccctctgtgcaccaccaacaccaaagagggctccaacatctgcctgacccggaccgacagaggctggtactgcgataatgccggctccgtctcattctttccacaagccgagacatgcaaggtgcagagcaaccgggtgttctgcgacaccatgaacagcctgaccctgccctccgaagtgaatctgtgcaacgtggacatcttcaaccctaagtacgactgcaagatcatgacctccaagaccgacgtgtccagctccgtgatcacaagcctgggcgccatcgtgtcctgctacggcaagaccaagtgcaccgccagcaacaagaaccggggcatcatcaagaccttcagcaacggctgcgactacgtgtccaacaagggggtggacaccgtgtctgtgggcaacaccctgtactacgtgaacaaacaggaaggcaagagcctgtacgtgaagggcgagcccatcatcaacttctacgaccccctggtgttccccagcgacgagttcgatgccagcatctcccaagtgaacgagaagatcaaccagagcctggccttcatcagaaagtccgatgagctgctgcacaatgtgaacgccggcaagtccaccaccaatatcatgatcaccacaatcatcatcgtgattatcgtgatcctgctgagcctgatcgccgtgggcctgctgctgtactgtatcatcaagttccaccggatccagggcaaggaccagaacgacaagaactccgagccctacatcctgacaaaccggcagtga

SEQ ID NO: 18 - DNA, 1728 bp, Artificial sequence
  Recombinant RSV F
atggaactgctgatcctgaaagccaacgctattactactatcctgaccgccgtgacattttgcttcgcatctggacagaacattactgaggaattctaccagtcaacatgcagcgccgtgtccaaaggatacctgagcgccctgcggaccggctggtatacatcagtgattactatcgagctgtccaacatcaaggaaaacaaatgtaatgggaccgacgcaaaggtgaaactgatcaagcaggagctggataagtacaaaaatgccgtgacagaactgcagctgctgatgcagtccacaccagcaactaacaatcgcgcccggagagagctgccccggttcatgaactataccctgaacaatgctaagaaaaccaatgtgacactgtccaagaaacgcaagaggcgcttcctgggatttctgctgggcgtggggtctgccatcgctagtggagtggccgtctgcaaagtcctgcacctggagggcgaagtgaacaagatcaaaagcgccctgctgtccactaacaaggcagtggtcagtctgtcaaatggcgtgtccgtcctgaccttcaaggtgctggacctgaaaaattatattgataagcagctgctgcctatcctgaacaaacagagctgctccatttctaatatcgagacagtgatcgaattccagcagaagaacaatagactgctggagattaccagagagttcagcgtgaacgccggcgtcaccacacccgtgtccacctacatgctgacaaatagtgagctgctgtcactgattaacgacatgcctatcaccaatgatcagaagaaactgatgtccaacaatgtgcagatcgtcagacagcagagttactcaatcatgtgcatcattaaggaggaagtcctggcctacgtggtccagctgccactgtatggcgtgatcgacaccccctgctggaaactgcatacatctcctctgtgcactaccaacacaaaggaaggaagtaatatctgcctgactcgaaccgaccggggatggtactgtgataacgcaggcagcgtgtccttctttccacaggccgagacctgcaaggtccagagcaacagggtgttctgtgacactatgaatagcctgaccctgccttccgaagtcaacctgtgcaatgtggacatctttaatccaaagtacgattgtaagatcatgactagcaagaccgatgtcagctcctctgtgattacttctctgggggccatcgtgagttgctacggaaagacaaaatgtactgccagcaacaaaaatcgcggcatcattaagaccttctccaacgggtgcgactatgtctctaacaagggcgtggatacagtgagtgtcgggaacactctgtactatgtcaataagcaggagggaaaaagcctgtacgtgaagggcgaacccatcattaacttctatgaccccctggtgttcccttccgacgagtttgatgcatctattagtcaggtgaacgaaaaaatcaatcagagtctggcctttattcggaagtcagatgagctgctgcacaacgtgaatgctggcaaatctacaactaacatcatgatcaccacaatcatcatcgtgattatcgtcattctgctgtcactgatcgctgtggggctgctgctgtactgtatcattaagttccaccggatccagggcaaggaccagaacgataaaaatagcgagccctacattctgaccaacagacag

SEQ ID NO: 19 - protein, 576 aa, Artificial sequence
  Recombinant RSV F
MELLILKANAITTILTAVTFCFASGQNITEEFYQSTCSAVSKGYLSALRTGWYTSVITIELSNIKENKCNGTDAKVKLIKQELDKYKNAVTELQLLMQSTPATNNRARRELPRFMNYTLNNAKKTNVTLSKKRKRRFLGFLLGVGSAIASGVAVCKVLHLEGEVNKIKSALLSTNKAVVSLSNGVSVLTSKVLDLKNYIDKQLLPIVNKQSCSISNIETVIEFQQKNNRLLEITREFSVNAGVTTPVSTYMLTNSELLSLINDMPITNDQKKLMSNNVQIVRQQSYSIMCIIKEEVLAYVVQLPLYGVIDTPCWKLHTSPLCTTNTKEGSNICLTRTDRGWYCDNAGSVSFFPQAETCKVQSNRVFCDTMNSLTLPSEVNLCNVDIFNPKYDCKIMTSKTDVSSSVITSLGAIVSCYGKTKCTASNKNRGIIKTFSNGCDYVSNKGVDTVSVGNTLYYVNKQEGKSLYVKGEPIINFYDPLVFPSDEFDASISQVNEKINQSLAFIRKSDELLHNVNAGKSTTNIMITTITIIIVMIIILVIINITIIVVIIKFHRIQGKDQNDKNSEPYILTNRQ

SEQ ID NO: 20 - DNA, 1731 bp, Artificial sequence
  Recombinant RSV F
atggaactgctgatcctgaaggccaacgccatcaccaccatcctgaccgccgtgaccttctgctttgccagcggccagaacatcaccgaggaattctaccagagcacctgtagcgccgtgtccaagggctacctgagcgccctgagaaccggctggtacaccagcgtgatcaccatcgagctgagcaacatcaaagaaaacaagtgcaacggcaccgacgccaaagtgaagctgatcaagcaggaactggacaagtacaagaatgccgtgaccgaactgcagctgctgatgcagagcacccccgccaccaacaaccgggccagaagagaactgcccagattcatgaactacaccctgaacaacgccaaaaagaccaacgtgaccctgagcaagaagcggaagcggcggttcctgggctttctgctgggagtgggaagcgccattgctagcggagtggccgtgtgcaaggtgctgcacctggaaggcgaagtgaacaagatcaagtccgccctgctgagcaccaacaaggccgtggtgtctctgagcaacggcgtgtccgtgctgaccagcaaggtgctggatctgaagaactacatcgacaaacagctgctgcccatcgtgaacaagcagagctgcagcatcagcaacatcgagacagtgatcgagttccagcagaagaacaaccggctgctggaaatcacccgcgagttcagcgtgaacgctggcgtgaccacccccgtgtccacctacatgctgaccaacagcgagctgctgtccctgatcaacgacatgcccatcaccaacgaccagaaaaagctgatgagcaacaacgtgcagatcgtgcggcagcagagctactccatcatgtgcatcatcaaagaagaggtgctggcctacgtggtgcagctgcctctgtacggcgtgatcgacaccccctgctggaagctgcacaccagccctctgtgcaccaccaacaccaaagagggctccaacatctgcctgacccggaccgacagaggctggtactgcgataatgccggctccgtctcattctttccacaagccgagacatgcaaggtgcagagcaaccgggtgttctgcgacaccatgaacagcctgaccctgccctccgaagtgaatctgtgcaacgtggacatcttcaaccctaagtacgactgcaagatcatgacctccaagaccgacgtgtccagctccgtgatcacaagcctgggcgccatcgtgtcctgctacggcaagaccaagtgcaccgccagcaacaagaaccggggcatcatcaagaccttcagcaacggctgcgactacgtgtccaacaagggggtggacaccgtgtctgtgggcaacaccctgtactacgtgaacaaacaggaaggcaagagcctgtacgtgaagggcgagcccatcatcaacttctacgaccccctggtgttccccagcgacgagttcgatgccagcatctcccaagtgaacgagaagatcaaccagagcctggccttcatcagaaagtccgatgagctgctgcacaatgtgaacgccggcaagtccaccaccaatatcatgatcaccacaatcaccatcatcattgtgatgattatcatcctcgtgatcatcaacatcacaatcatcgtcgtgattattaagttccaccggatccagggcaaggaccagaacgacaagaactccgagccctacatcctgacaaaccggcagtga

SEQ ID NO: 21 - protein, 576 aa, Artificial sequence
  Recombinant RSV F
MELLILKANAITTILTAVTFCFASGQNITEEFYQSTCSAVSKGYLSALRTGWYTSVITIELSNIKENKCNGTDAKVKLIKQELDKYKNAVTELQLLMQSTPATNNRARRELPRFMNYTLNNAKKTNVTLSKKRKRRFLGFLLGVGSAIASGVAVCKVLHLEGEVNKIKSALLSTNKAVVSLSNGVSVLTFKVLDLKNYIDKQLLPILNKQSCSISNIETVIEFQQKNNRLLEITREFSVNAGVTTPVSTYMLTNSELLSLINDMPITNDQKKLMSNNVQIVRQQSYSIMCIIKEEVLAYVVQLPLYGVIDTPCWKLHTSPLCTTNTKEGSNICLTRTDRGWYCDNAGSVSFFPQAETCKVQSNRVFCDTMNSLTLPSEVNLCNVDIFNPKYDCKIMTSKTDVSSSVITSLGAIVSCYGKTKCTASNKNRGIIKTFSNGCDYVSNKGVDTVSVGNTLYYVNKQEGKSLYVKGEPIINFYDPLVFPSDEFDASISQVNEKINQSLAFIRKSDELLHNVNAGKSTTNIMITTITIIIVMIIILVIINITIIVVIIKFHRIQGKDQNDKNSEPYILTNRQ

SEQ ID NO: 22 - DNA, 1731 bp, Artificial sequence
  Recombinant RSV F
atggaactgctgatcctgaaggccaacgccatcaccaccatcctgaccgccgtgaccttctgctttgccagcggccagaacatcaccgaggaattctaccagagcacctgtagcgccgtgtccaagggctacctgagcgccctgagaaccggctggtacaccagcgtgatcaccatcgagctgagcaacatcaaagaaaacaagtgcaacggcaccgacgccaaagtgaagctgatcaagcaggaactggacaagtacaagaatgccgtgaccgaactgcagctgctgatgcagagcacccccgccaccaacaaccgggccagaagagaactgcccagattcatgaactacaccctgaacaacgccaaaaagaccaacgtgaccctgagcaagaagcggaagcggcggttcctgggctttctgctgggagtgggaagcgccattgctagcggagtggccgtgtgcaaggtgctgcacctggaaggcgaagtgaacaagatcaagtccgccctgctgagcaccaacaaggccgtggtgtctctgagcaacggcgtgtccgtgctgaccttcaaggtgctggatctgaagaactacatcgacaaacagctgctgcccatcttgaacaagcagagctgcagcatcagcaacatcgagacagtgatcgagttccagcagaagaacaaccggctgctggaaatcacccgcgagttcagcgtgaacgctggcgtgaccacccccgtgtccacctacatgctgaccaacagcgagctgctgtccctgatcaacgacatgcccatcaccaacgaccagaaaaagctgatgagcaacaacgtgcagatcgtgcggcagcagagctactccatcatgtgcatcatcaaagaagaggtgctggcctacgtggtgcagctgcctctgtacggcgtgatcgacaccccctgctggaagctgcacaccagccctctgtgcaccaccaacaccaaagagggctccaacatctgcctgacccggaccgacagaggctggtactgcgataatgccggctccgtctcattctttccacaagccgagacatgcaaggtgcagagcaaccgggtgttctgcgacaccatgaacagcctgaccctgccctccgaagtgaatctgtgcaacgtggacatcttcaaccctaagtacgactgcaagatcatgacctccaagaccgacgtgtccagctccgtgatcacaagcctgggcgccatcgtgtcctgctacggcaagaccaagtgcaccgccagcaacaagaaccggggcatcatcaagaccttcagcaacggctgcgactacgtgtccaacaagggggtggacaccgtgtctgtgggcaacaccctgtactacgtgaacaaacaggaaggcaagagcctgtacgtgaagggcgagcccatcatcaacttctacgaccccctggtgttccccagcgacgagttcgatgccagcatctcccaagtgaacgagaagatcaaccagagcctggccttcatcagaaagtccgatgagctgctgcacaatgtgaacgccggcaagtccaccaccaatatcatgatcaccacaatcaccatcatcattgtgatgattatcatcctcgtgatcatcaacatcacaatcatcgtcgtgattattaagttccaccggatccagggcaaggaccagaacgacaagaactccgagccctacatcctgacaaaccggcagtga

SEQ ID NO: 23 - DNA, 1731 bp, Artificial sequence
  Recombinant RSV F
atggaactgctgatcctgaaagccaacgctattactactatcctgaccgccgtgacattttgcttcgcatctggacagaacattactgaggaattctaccagtcaacatgcagcgccgtgtccaaaggatacctgagcgccctgcggaccggctggtatacatcagtgattactatcgagctgtccaacatcaaggaaaacaaatgtaatgggaccgacgcaaaggtgaaactgatcaagcaggagctggataagtacaaaaatgccgtgacagaactgcagctgctgatgcagtccacaccagcaactaacaatcgcgcccggagagagctgccccggttcatgaactataccctgaacaatgctaagaaaaccaatgtgacactgtccaagaaacgcaagaggcgcttcctgggatttctgctgggcgtggggtctgccatcgctagtggagtggccgtctgcaaagtcctgcacctggagggcgaagtgaacaagatcaaaagcgccctgctgtccactaacaaggcagtggtcagtctgtcaaatggcgtgtccgtcctgaccttcaaggtgctggacctgaaaaattatattgataagcagctgctgcctatcctgaacaaacagagctgctccatttctaatatcgagacagtgatcgaattccagcagaagaacaatagactgctggagattaccagagagttcagcgtgaacgccggcgtcaccacacccgtgtccacctacatgctgacaaatagtgagctgctgtcactgattaacgacatgcctatcaccaatgatcagaagaaactgatgtccaacaatgtgcagatcgtcagacagcagagttactcaatcatgtgcatcattaaggaggaagtcctggcctacgtggtccagctgccactgtatggcgtgatcgacaccccctgctggaaactgcatacatctcctctgtgcactaccaacacaaaggaaggaagtaatatctgcctgactcgaaccgaccggggatggtactgtgataacgcaggcagcgtgtccttctttccacaggccgagacctgcaaggtccagagcaacagggtgttctgtgacactatgaatagcctgaccctgccttccgaagtcaacctgtgcaatgtggacatctttaatccaaagtacgattgtaagatcatgactagcaagaccgatgtcagctcctctgtgattacttctctgggggccatcgtgagttgctacggaaagacaaaatgtactgccagcaacaaaaatcgcggcatcattaagaccttctccaacgggtgcgactatgtctctaacaagggcgtggatacagtgagtgtcgggaacactctgtactatgtcaataagcaggagggaaaaagcctgtacgtgaagggcgaacccatcattaacttctatgaccccctggtgttcccttccgacgagtttgatgcatctattagtcaggtgaacgaaaaaatcaatcagagtctggcctttattcggaagtcagatgagctgctgcacaacgtgaatgctggcaaatctacaactaacatcatgatcaccacaatcaccatcattatcgtgatgattatcattctggtcatcattaacatcacaatcattgtggtcatcattaagttccaccggattcagggcaaggaccagaacgataaaaatagcgagccctacatcctgaccaatagacagtga

SEQ ID NO: 24 - protein, 524 aa, Human parainfluenza virus 1
MAGLLSTFDTFSSRRSESINKSGGGAIIPGQRSTVSVFTLGPSVTDDADKLLIATTFLAHSLDTDKQHSQRGGFLVSLLAMAYSSPELYLTTNGVNADVKYVIYNIERDPKRTKTDGFIVKTRDMEYERTTEWLFGPMINKNPLFQGQRENADLEALLQTYGYPACLGAIIVQVWIVLVKAITSSAGLRKGFFNRLEAFRQDGTVKSALVFTGDTVEGIGAVMRSQQSLVSLMVETLVTMNTSRSDLTTLEKNIQIVGNYIRDAGLASFMNTIKYGVETKMAALTLSNLRPDINKLRSLVDIYLSKGARAPFICILRDPVHGDFAPGNYPALWSYAMGVAVVQNKAMQQYVTGRTYLDMEMFLLGQAVAKDADSKISSALEEELGVTDTAKERLRHHLTNLSGGDGAYHKPTGGGAIEVAIDHTDITFGVEDTADRDNKNWTNDSNERWMNHSISNHTITIRGAEELEEETNDEDITDIENKIARRLADRKQRLSQANNKRDTSSDADYENDDDATAAAGIGGI

SEQ ID NO: 25 - protein, 568 aa, Human parainfluenza virus 1
MDQDAFFFERDPEAEGEAPRKQESLSDVIGLLDVVLSYKPTEIGEDRSWLHGIIDNPKENKPSCKADDNNKDRAISTSTQDHRSSEESGISRRTSESKTETHARILDQQGIHRASRRGTSPNPLPENMGNERNTRIDEDSPNERRHQRSVLTDEDRKMAENSNKREEDQVEGFPEEVRRSTPLSDDGEGRTNNNGRSMETSSTHSTRITDVITNPSPELEDAVLQRNKRRPTTIKRNQTRSERTQSSELHKSTSENSSNLEDHNTKTSPKVPPSKNEESAATPKNNHNHRKTRYTTNNANNNTKSPPTPEHDATANEEETSNTSVDEMAKLLVSLGVMKSQHEFELSRSASHVFAKRMLKSANYKEMTFNLCGMLISVEKSLENKVEENRTLLKQIQEEINSSRDLHKRFSEYQKEQNSLMMANLSTLHIITDRGGKTGNPSDTTRSPSVFTKGKDNKVKKTRFDPSMEALGGQEFKPDLIREDELRDDIKNPVLEENNNEPQASNASRLIPSTEKHTLHSLKLVIENSPLSRVEKKAYIKSLYKCRTNQEVKNVMELFEEDIDSLTN

SEQ ID NO: 26 - protein, 204 aa, Human parainfluenza virus 1
MPSFLRGILKPKERHHENKNHSQMSSDSLTSSYPTSPQKLEKTEAGSMVSSTTQKKTSHHAKPTITTKTEQSQRRPKIIDQVRRVESLGEQVSQKQRHMLESLINKVYTGPLGEELVQTLYLRIWAMKETPESTKILQMREDIRDQYLRMKTERWLRTLIRGKKTKLRDFQKRYEEVHPYLMMERVEQIIMEEAWKLAAHIVQE

SEQ ID NO: 27 - protein, 348 aa, Human parainfluenza virus 1
MAETYRFPRFSHEENGTVEPLPLKTGPDKKAIPHIRIVKVGDPPKHGVRYLDVLLLGFFETPKQGPLSGSISDLTESTSYSICGSGSLPIGIAKYYGTDQELLKACIDLKITVRRTVRSGEMIVYMVDSIHAPLLPWSSRLRQGMIYNANKVALAPQCLPVDKDIRFRVVFVNGTSLGTITIAKVPKTLADLALPNSISVNLLVTLRAGVSTEQKGILPVLDDDGEKKLNFMVHLGIIRRKVGKIYSVEYCKNKIEKMKLIFSLGLVGGISFHVHATGTLSKTLMSQLAWKKAVCYPLMDVNPHMNLVIWAASVEITSVDAVFQPAIPKEFRYYPNVVAKSIGKIRRI

SEQ ID NO: 28 - protein, 555 aa, Human parainfluenza virus 1
MQKSEILFLVYSSLLLSSSLCQIPVEKLSNVGVIINEGKLLKIAGSYESRYIVLSLVPSIDLQDGCGTTQIIQYKNLLNRLLIPLKDALDLQESLITITNDTTVTNDNPQTRFFGAVIGTIALGVATAAQITAGIALAEAREARKDIALIKDSIVKTHNSVELIQRGIGEQIIALKTLQDFVNDEIRPAIGELRCETTALKLGIKLTQHYSELATAFSSNLGTIGEKSLTLQALSSLYSANITEILSTTKKDKSDIYDIIYTEQVKGTVIDVDLEKYMVTLLVKIPILSEIPGVLIYRASSISYNIEGEEWHVAIPNYIINKASSLGGADVTNCIESKLAYICPRDPTQLIPDNQQKCILGDVSKCPVTKVINNLVPKFAFINGGVVANCIASTCTCGTNRIPVNQDRSRGVTFLTYTNCGLIGINGIELYANKRGRDTTWGNQIIKVGPAVSIRPVDISLNLASATNFLEESKTELMKARAIISAVGGWHNTESTQIIMIIIVCILIIIICGILYYLYRVRRLLVMINSTHNSPVNAYTLESRMRNPYMGNNSN

SEQ ID NO: 29 - protein, 575 aa, Human parainfluenza virus 1
MAEKGKTNSSYWSTTRNDNSTVNTHINTPAGRTHIWLLIATTMHTVLSFIIMILCIDLIIKQDTCMKTNIMTVSSMNESAKIIKETITELIRQEVISRTINIQSSVQSGIPILLNKQSRDLTQLIEKSCNRQELAQICENTIAIHHADGISPLDPHDFWRCPVGEPLLSNNPNISLLPGPSLLSGSTTISGCVRLPSLSIGDAIYAYSSNLITQGCADIGKSYQVLQLGYISLNSDMYPDLNPVISHTYDINDNRKSCSVIAAGTRGYQLCSLPTVNETTDYSSEGIEDLVFDILDLKGKTKSHRYKNEDITFDHPFSAMYPSVGSGIKIENTLIFLGYGGLTTPLQGDTKCVINRCTNVNQSVCNDALKITWLKKRQVVNVLIRINNYLSDRPKIVVETIPITQNYLGAEGRLLKLGKKIYIYTRSSGWHSNLQIGSLDINNPMTIKWAPHEVLSRPGNQDCNWYNRCPRECISGVYTDAYPLSPDAVNVATTTLYANTSRVNPTIMYSNTSEIINMLRLKNVQLEAAYTTTSCITHFGKGYCFHIVEINQTSLNTLQPMLFKTSIPKICKITS

SEQ ID NO: 30 - protein, 2223 aa, Human parainfluenza virus 1
MDKQESTQNSSDILYPECHLNSPIVKSKIAQLHVLLDINQPYDLKDNSIINITKYKIRNGGLSPRQIKIRSLGKILKQEIKDIDRYTFEPYPIFSLELLRLDIPEICDKIRSIFSVSDRLIRELSSGFQELWLNILRQLGCVEGKEGFDSLKDVDIIPDITDKYNKNTWYRPFLTWFSIKYDMRWMQKNKSGNHLDVSNSHNFLDCKSYILIIYRDLVIIINKLKLTGYVLTPELVLMYCDVVEGRWNMSSAGRLDKRSSKITCKGEELWELIDSLFPNLGEDVYNIISLLEPLSLALIQLDDPVTNLKGAFMRHVLTELHTILIKDNIYTDSEADSIMESLIKIFRETSIDEKAEIFSFFRTFGHPSLEAITAADKVRTHMYSSKKIILKTLYECHAIFCAIIINGYRERHGGQWPPCEFPNHVCLELKNAQGSNSAISYECAVDNYSSFIGFKFLKFIEPQLDEDLTIYMKDKALSPRKAAWDSVYPDSNLYYKVPESEETRRLIEVFINDNNFNPADIINYVESGEWLNDDSFNISYSLKEKEIKQEGRLFAKMTYKMRAVQVLAETLLAKGVGELFSENGMVKGEIDLLKRLTTLSVSGVPRSNSVYNNPILHEKLIKNMNKCNSNGYWDERKKSKNEFKAADSSTEGYETLSCFLTTDLKKYCLNWRFESTALFGQRCNEIFGFKTFFNWMHPILEKSTIYVGDPYCPVPDRMHKELQDHDDTGIFIHNPRGGIEGYCQKLWTLISISAIHLAAVKVGVRVSAMVQGDNQAIAVTSRVPVTQTYKQKKTHVYEEITRYFGALREVMFDIGHELKLNETIISSKMFVYSKRIYYDGKILPQCLKALTRCVFWSETLVDENRSACSNIATSIAKAIENGYSPILGYCIALFKTCQQVCISLGMTINPTITSTIKDQYFKGKNWLRCAILIPANIGGFNYMSTARCFVRNIGDPAVAALADLKRFIKAGLLDKQVLYRVMNQEPGDSSFLDWASDPYSCNLPHSQSITTIIKNVTARSVLQESPNPLLSGLFSESSSEEDLNLASFLMDRKAILPRVAHEILDNSLTGVREAIAGMLDTTKSLVRASVRRGGLSYSILRRLINYDLLQYETLTRTLRKPVKDNIEYEYMCSVELAIGLRQKMWFHLTYGRPIHGLETPDPLELLRGSFIEGSEICKFCRSEGNNPMYTWFYLPDNIDLDTLSNGSPAIRIPYFGSATDERSEAQLGYVKNLSKPAKAAIRIAMVYTWAYGTDEISWMEAALIAQTRANLSLENLKLLTPVSTSTNLSHRLRDTATQMKFSSATLVRASRFITISNDNMALKEAGESKDTNLVYQQIMLTGLSLFEFNMRYKQGSLSKPMILHLHLNNKCCIIESPQELNIPPRSTLDLEITQENNKLIYDPDPLKDIDLELFSKVRDVVHTIDMNYWSDDEIIRATSICTAMTIADTMSQLDRDNLKEMIALINDDDINSLITEFMVIDIPLFCSTFGGILINQFAYSLYGLNVRGRDEIWGYVIRIIKDTSHAVLKVLSNALSHPKIFKRFWDAGVVEPVYGPNLSNQDKILLAISVCEYSVDLFMRDWQEGIPLEIFICDNDPNIAEMRKLSFLARHLAYLCSLAEIAKEGPKLESMTSLERLESLKEYLELTFLDDPILRYSQLTGLVIKIFPSTLTYIRKSSIKVLRVRGIGIPEVLEDWDPDADSMLLDNITAEVQHNIPLKKNERTPFWGLRVSKSQVLRLRGYEEIKREERGRSGVGLTLPFDGRYLSHQLRLFGINSTSCLKALELTYLLNPLVNKDKDRLYLGEGAGAMLSCYDATLGPCMNYYNSGVNSCDLNGQRELNIYPSEVALVGKKLNNVTSLCQRVKVLFNGNPGSTWIGNDECETLIWNELQNNSIGFIHCDMEGGEHKCDQVVLHEHYSVIRIAYLVGDKDVILVSKIAPRLGTDWTKQLSLYLRYWRDVSLIVLKTSNPASTEMYLISKDPKSDIIEDSNTVLANLLPLSKEDSIKIEKWILVEKAKVHDWIVRELKEGSASSGMLRPYHQALQIFGFEPNLNKLCRDFLSTLNIVDTKNCIITFDRVLRDTIFEWTRIKDADKKLRLTGKYDLYPLRDSGKLKVISRRLVISWIALSMSTRLVTGSFPDIKFESRLQLGIVSISSREIKNLRVISKIVIDKFEDIIHSVTYRFLTKEIKILMKILGAVKLFGARQSTSADITNIDTSDSIQ

SEQ ID NO: 31 - protein, 59 aa, Human parainfluenza virus 1
QIIMIIIVCILIIIICGILYYLYRVRRLLVMINSTHNSPVNAYTLESRMRNPYMGNNSN

SEQ ID NO: 32 - protein, 543 aa, Human parainfluenza virus 2
MSSVLKTFERFTIQQELQEQSEDTPIPLETIRPTIRVFVINNNDPIVRSRLLFFNLRIIMSNTAREGHRAGALLSLLSLPSAAMSNHIKLAMHSPEASIDRVEITGFENNSFRVIPDARSTMSRGEVLAFEALAEDIPDTLNHQTPFVNNDVEDDIFDETEKFLDVCYSVLMQAWIVTCKCMTAPDQPPVSVAKRMAKYQQQGRINARYVLQPEAQRLIQNAIRKSMVVRHFMTYELQLSQSRSLLANRYYAMVGDIGKYIEHSGMGGFFLTLKYGLGTRWPTLALAAFSGELQKLKALMLHYQSLGPMAKYMALLESPKLMDFVPSEYPLVYSYAMGIGTVLDTNMRNYAYGRSYLNPQYFQLGVETARKQQGAVDNRTAEDLGMTAADKADLTATISKLSLSQLPRGRQPISDPFAGANDRETGGQATDTPVYNFNPINNRRYDNYDSDSEDRIDNDQDQAIRENRGEPGQPNNQTSENQQRLNLPVPQRTSGMSSEEFQHSMNQYIRAMHEQYRGSQDDDANDATDGNDISLELVGDFDS

SEQ ID NO: 33 - protein, 395 aa, Human parainfluenza virus 2
MAEEPTYTTEQVDELIHAGLGTVDFFLSRPIDAQSSLGKGSIPPGVTAVLTNAAEAKSKPVAAGPVKPRRKKVISNTTPYTIADNIPPEKLPINTPIPNPLLPLARPHGKMTDIDIVTGNITEGSYKGVELAKLGKQTLLTRFTSNEPVSSAGSAQDPNFKRGGELIEKEQEATIGENGVLHGSEIRSKSSSGVIPGVPQSRLQLASSPAHVDPAPASAENVKEIIELLKGLDLRLQTVEGKVDKILATSATIINLKNEMTSLKASVATVEGMITTIKIMDPSTPTNVPVEEIRKSLHNVPVVIAGPTSGGFTAEGSDMISMDELARPTLSSTKKITRKPESKKDLTGIKLTLMQLANDCISRPDTKTEFVTKIQAATTESQLNEIKRSIIRSAI

SEQ ID NO: 34 - protein, 225 aa, Human parainfluenza virus 2
MAEEPTYTTEQVDELIHAGLGTVDFFLSRPIDAQSSLGKGSIPPGVTAVLTNAAEAKSKPVAAGPVKPRRKKVISNTTPYTIADNIPPEKLPINTPIPNPLLPLARPHGKMTDIDIVTGNITEGSYKGVELAKLGKQTLLTRFTSNEPVSSAGSAQDPNFKRGGANRERARGNHRREWSIAWVGDQVKVFEWCNPRCAPVTASARKFTCTCGSCPSICGECEGDH

SEQ ID NO: 35 - protein, 377 aa, Human parainfluenza virus 2
MPIISLPADPTSPSQSLTPFPIQLDTKDGKAGKLLKQIRIRYLNEPNSRHTPITFINTYGFVYARDTSGGIHSEISSDLAAGSITACMMTLGPGPNIQNANLVLRSLNEFYVKVKKTSSQREEAVFELVNIPTLLREHALCKRKTLVCSAEKFLKNPSKLQAGFEYVYIPTFVSITYSPRNLNYQVARPILKFRSRFVYSIHLELILRLLCKSDSPLMKSYNADRTGRGCLASVWIHVCNILKNKSIKQQGRESYFIAKCMSMQLQVSIADLWGPTIIIKSLGHIPKTALPFFSKDGIACHPLQDVSPTLTKSLWSVGCEIESAKLILQESDINELMGHQDLITDKIAIRSGQRTFERSKFSPFKKYASIPNLEAIN

SEQ ID NO: 36 - protein, 551 aa, Human parainfluenza virus 2
MHHLHPMIVCIFVMYTGIVGSDAIAGDQLLNVGVIQSKIRSLMYYTDGGASFIVVKLLPNLPPSNGTCNITSLDAYNVTLFKLLTPLIENLSKISAVTDTKPRRERFAGVVIGLAALGVATAAQITAAVAIVKANANAAAINNLASSIQSTNKAVSDVITASRTIATAVQAIQDHINGAIVNGITSASCRAHDALIGSILNLYLTELTTIFHNQITNPALTPLSIQALRILLGSTLPIVIESKLNTKLNTAELLSSGLLTGQIISISPMYMQMLIQINVPTFIMQPGAKVIDLIAISANHKLQEVVVQVPNRILEYANELQNYPANDCVVTPNSVFCRYNEGSPIPESQYQCLRGNLNSCTFTPIIGNFLKRFAFANGVLYANCKSLLCKCADPPHVVSQDDNQGISIIDIKRCSEMMLDTFSFRITSTFNATYVTDFSMINANIVHLSPLDLSNQINSINKSLKSAEDWIADSNFFANQARTAKTLYSLSAIALILSVITLVVVGLLIAYIIKLVSQIHQFRALAATTMFHRENPAVFSKNNHGNIYGIS

SEQ ID NO: 37 - protein, 571 aa, Human parainfluenza virus 2
MEDYSNLSLKSIPKRTCRIIFRTATILGICTLIVLCSSILHEIIHLDVSSGLMNSDESQQGIIQPIIESLKSLIALANQILYNVAIVIPLKIDSIETVILSALKDMHTGSMSNANCTPGNLLLHDAAYINGINKFLVLESYNGTPKYGPLLNIPSFIPSATSPHGCTRIPSFSLIKTHWCYTHNVMLGDCLDFTASNQYLSMGIIQQSAAGFPIFRTMKTIYLSDGINRKSCSVTAIPGGCVLYCYVATRSEKEDYATTDLAELRLAFYYYNDTFIERVISLPNTTGQWATINPAVGSGIYHLGFILFPVYGGLINGTTSYNEQSSRYFIPKHPNITCAGNSSKQAAIARSSYVIRYHSNRLIQSAVLICPLSDMHTEECNLVMFNNSQVMMGAEGRLYVIGNNLYYYQRSSSWWSASLFYRINTDFSKGIPPIIEAQWVPSYQVPRPGVMPCNATSFCPANCITGVYADVWPLNDPELMSRNALNPNYRFAGAFLKNESNRTNPTFYTASANSLLNTTGFNNTNHKAAYTSSTCFKNTGTQKIYCLIIIEMGSSLLGEFQIIPFLRELML

SEQ ID NO: 38 - protein, 2263 aa, Human parainfluenza virus 2
MAASSEILLPEVHLNSPIVKHKLIYYLLLGHFPHDLDISEISPLHNNDWDQIAREESNLAERLGVAKSELIKRVPAFRATRWRSHAAVLIWPSCIPFLVKFLPHSKLQPIEQWYKLINASCNTISDSIDRCMENISIKLTGKNNLFSRSRGTAGAGKNSKITLNDIQSIWESNKWQPNVSLWLTIKYQMRQLIMHQSSRQPTDLVHIVDTRSGLIVITPELVICFDRLNNVLMYFTFEMTLMVSDMFEGRMNVAALCTISHYLSPLGPRIDRLFSIVDELAQLLGDTVYKIIASLESLVYGCLQLKDPVVELTGSFHSFITQEIIDILIGSKALDKDESITVTTQLLDIFSNLSPDLIAEMLCLMRLWGHPTLTAAQAAGKVRESMCAGKLLDFPTIMKTLAFFHTILINGYRRKKNGMWPPLILPKNASKSLIEFQHDNAEISYEYTLKHWKEISLIEFRKCFDFDPGEELSIFMKDKAISAPKSDWMSVFRRSLIKQRHQRHHIPMPNPFNRRLLLNFLEDDSFDPVAELQYVTSGEYLRDDTFCASYSLKEKEIKPDGRIFAKLTNRMRSCQVIAEAILANHAGTLMKENGVVLNQLSLTKSLLTMSQIGIISEKAKRYTRDNISSQGFHTIKTDSKNKKKSKIASSYLTDPDDTFELSACFITTDLAKYCLQWRYQTIIHFARTLNRMYGVPHLFEWIHLRLIRSTLYVGDPFNPPATTDAFDLDKVLNGDIFIVSPKGGIEGLCQKMWTMISISVIILSSAESKTRVMSMVQGDNQAIAVTTRVPRSLPSVQKKELAYAASKLFFERLRANNYGLGHQLKAQETIISSTFFIYSKRVFYQGRILTQALKNASKLCLTADVLGECTQASCSNSATTIMRLTENGVEKDTCYKLNIYQSIRQLTYDLIFPQYSIPGETISEIFLQHPRLISRIVLLPSQLGGLNYLACSRLFNRNIGDPLGTAVADLKRLIKCGALESWILYNLLARKPGKGSWATLAADPYSLNQEYLYPPTTILKRHTQNTLMEICRNPMLKGVFTDNAKEEENLLAKFLLDRDIVLPRVAHIIIDQSSIGRKKQIQGFFDTTRTIMRRSFEIKPLSTKKTLSVIEYNTNYLSYNYPVILNPLPIPGYLNYITDQTCSIDISRSLRKLSWSSLLNGRTLEGLETPDPIEVVNGSLIVGTGDCDFCMQGDDKFTWFFLPMGIIIDGNPETNPPIRVPYIGSRTEERRVASMAYIKGATHSLKAALRGAGVYIWAFGDTVVNWNDALDIANTRVKISLEQLQTLTPLPTSANITHRLDDGATTLKFTPASSYAFSSYTHISNDQQYLEIDQRVVDSNIIYQQLMITGLGIIETYHNPPIRTSTQEITLHLHTSSSCCVRSVDGCLICESNGEVPQITVPYTNSFVYDPDPLADYEIAHLDYLSYQAKIGSTDYYSLTDKIDLLAHLTAKQMINSIIGLDETVSIVNDAVILSDYTNNWISECSYTKIDLVFKLMAWNFLLELAFQMYYLRISSWTNIFDYTYMTLRRIPGTALNNIAATISHPKLLRRAMNLDIITPIHAPYLASLDYVKLSIDAIQWGVKQVLADLSNGIDLEILILSEDSMEISDRAMNLIARKLTLLALVKGENYTFPKIKGMPPEEKCLVLTEYLAMCYQNTHHLDPDLQKYLYNLTNPKLTAFPSNNFYLTRKILNQIRESDEGQYIITSYYESFEQLETDIILHSTLTAPYDNSETLTKFDLSLDIFPHPESLEKYPLPVDHDSQSAISTLIPGPPSHHVLRPLGVSSTAWYKGISYCRYLETQKIQTGDHLYLAEGSGASMSLLELLFPGDTVYYNSLFSSGENPPQRNYAPLPTQFVQSVPYKLWQADLADDSNLIKDFVPLWNGNGAVTDLSTKDAVAFIIHKVGAEKASLVHIDLESTANINQQTLSRSQIHSLIIATTVLKRGGILVYKTSWLPFSRFSQLASLLWCFFDRIHLIRSSYSDPHSHEVYLVCRLAADFRTIGFSAALVTATTLHNDGFTTIHPDVVCSYWQHHLENVGRVEKVIDEILDGLATNFFAGDNGLILRCGGTPSSRKWLEIDQLASFDSVQDALVTLITIHLKEIIEVQSSHTEDYTSLLFTPYNIGAAGKVRTIIKLILERSLMYTVRNWLVLPSSIRDSVRQDLELGSFRLMSILSEQTFLKKTPTKKYLLDQLTRTYISTFFNSHSVLPLHRPYQKQIWKALGSVIYCSETVDIPLIRDIQIEDINDFEDIERGIDGEEL

SEQ ID NO: 39 - protein, 66 aa, Human parainfluenza virus 2
TLYSLSAIALILSVITLVVVGLLIAYIIKLVSQIHQFRALAATTMFHRENPAVFSKNNHGNIYGIS

SEQ ID NO: 40 - protein, 515 aa, Human parainfluenza virus 3
MLSLFDTFNARRQENITKSAGGAIIPGQKNTVSIFALGPTITDDNEKMTLALLFLSHSLDNEKQHAQRAGFLVSLLSMAYANPELYLTTNGSNADVKYVIYMIEKDLKRQKYGGFVVKTREMIYEKTTDWIFGSDLDYDQETMLQNGRNNSTIEDLVHTFGYPSCLGALIIQIWIVLVKAITSISGLRKGFFTRLEAFRQDGTVQAGLVLSGDTVDQIGSIMRSQQSLVTLMVETLITMNTSRNDLTTIEKNIQIVGNYIRDAGLASFFNTIRYGIETRMAALTLSTLRPDINRLKALMELYLSKGPRAPFICILRDPIHGEFAPGNYPAIWSYAMGVAVVQNRAMQQYVTGRSYLDIDMFQLGQAVARDAEAQMSSTLEDELGVTHESKESLKRHIRNINSSETSFHKPTGGSAIEMAIDEEPEQFEHRADQEQNGEPQSSIIQYAWAEGNRSDDQTEQATESDNIKTEQQNIRDRLNKRLNDKKKQSSQPPTNPTNRTNQDEIDDLFNAFGSN

SEQ ID NO: 41 - protein, 603 aa, Human parainfluenza virus 3
MESDAKNYQIMDSWEEESRDKSTNISSALNIIEFILSTDPQEDLSENDTINTRTQQLSATICQPEIKPTETSEKDSGSTDKNRQSGSSHECTTEAKDRNIDQETVQRGPGRRSSSDSRAETVVSGGIPRSITDSKNGTQNTEDIDLNEIRKMDKDSIEGKMRQSANVPSEISGSDDIFTTEQSRNSDHGRSLESISTPDTRSISVVTAATPDDEEEILMKNSRTKKSSSTHQEDDKRIKKGGKGKDWFKKSKDTDNQIPTSDYRSTSKGQKKISKTTTTNTDTKGQTEIQTESSETQSSSWNLIIDNNTDRNEQTSTTPPTTTSRSTYTKESIRTNSESKPKTQKTNGKERKDTEESNRFTERAITLLQNLGVIQSTSKLDLYQDKRVVCVANVLNNVDTASKIDFLAGLVIGVSMDNDTKLTQIQNEMLNLKADLKKMDESHRRLIENQREQLSLITSLISNLKIMTERGGKKDQNESNERVSMIKTKLKEEKIKKTRFDPLMEAQGIDKNIPDLYRHAGDTLENDVQVKSEILSSYNESNATRLIPKKVSSTMRSLVAVINNSNLSQSTKQSYINELKRCKNDEEVSELMDMFNEDVNNCQ

SEQ ID NO: 42 - protein, 353 aa, Human parainfluenza virus 3
MSITNSAIYTFPESSFSENGHIEPLPLKVNEQRKAVPHIRVAKIGNPPKHGSRYLDVFLLGFFEMERIKDKYGSVNDLDSDPSYKVCGSGSLPIGLAKYTGNDQELLQAATKLDIEVRRTVKAKEMVVYTVQNIKPELYPWSNRLRKGMLFDANKVALAPQCLPLDRSIKFRVIFVNCTAIGSITLFKIPKSMASLSLPNTISINLQVHIKTGVQTDSKGIVQILDEKGEKSLNFMVHLGLIKRKVGRMYSVEYCKQKIEKMRLIFSLGLVGGISLHVNATGSISKTLASQLVFKREICYPLMDLNPHLNLVIWASSVEITRVDAIFQPSLPGEFRYYPNIIAKGVGKIKQWN

SEQ ID NO: 43 - protein, 539 aa, Human parainfluenza virus 3
MPTSILLIITTMIMASFCQIDITKLQHVGVLVNSPKGMKISQNFETRYLILSLIPKIEDSNSCGDQQIKQYKKLLDRLIIPLYDGLRLQKDVIVTNQESNENTDPRTKRFFGGVIGTIALGVATSAQITAAVALVEAKQARSDIEKLKEAIRDTNKAVQSVQSSIGNLIVAIKSVQDYVNKEIVPSIARLGCEAAGLQLGIALTQHYSELTNIFGDNIGSLQEKGIKLQGIASLYRTNITEIFTTSTVDKYDIYDLLFTESIKVRVIDVDLNDYSITLQVRLPLLTRLLNTQIYKVDSISYNIQNREWYIPLPSHIMTKGAFLGGADVKECIEAFSSYICPSDPGFVLNHEIESCLSGNISQCPRTTVTSDIVPRYAFVNGGVVANCITTTCTCNGIGNRINQPPDQGVKIITHKECSTIGINGMLFNTNKEGTLAFYTPNDITLNNSVALDPIDISIELNKAKSDLEESKEWIRRSNQKLDSIGNWHQSSTTIIIILIMIIILFIINITIITIAIKYYRIQKRNRVDQNDKPYVLTNK

SEQ ID NO: 44 - protein, 572 aa, Human parainfluenza virus 3
MEYWKHTNHGKDAGNELETSMATHGNKLTNKIIYILWTIILVLLSIVFIIVLINSIKSEKAHESLLQDINNEFMEITEKIQMASDNTNDLIQSGVNTRLLTIQSHVQNYIPISLTQQMSDLRKFISEITIRNDNQEVLPQRITHDVGIKPLNPDDFWRCTSGLPSLMKTPKIRLMPGPGLLAMPTTVDGCVRTPSLVINDLIYAYTSNLITRGCQDIGKSYQVLQIGIITVNSDLVPDLNPRISHTFNINDNRKSCSLALLNTDVYQLCSTPKVDERSDYASSGIEDIVLDIVNYDGSISTTRFKNNNISFDQPYAALYPSVGPGIYYKGKIIFLGYGGLEHPINENVICNTTGCPGKTQRDCNQASHSPWFSDRRMVNSIIVVDKGLNSIPKLKVWTISMRQNYWGSEGRLLLLGNKIYIYTRSTSWHSKLQLGIIDITDYSDIRIKWTWHNVLSRPGNNECPWGHSCPDGCITGVYTDAYPLNPTGSIVSSVILDSQKSRVNPVITYSTATERVNELAILNRTLSAGYTTTSCITHYNKGYCFHIVEINHKSLNTFQPMLFKTEIPKSCS

SEQ ID NO: 45 - protein, 2233 aa, Human parainfluenza virus 3
MDTESNNGTVSDILYPECHLNSPIVKGKIAQLHTIMSLPQPYDMDDDSILVITRQKIKLNKLDKRQRSIRRLKLILTEKVNDLGKYTFIRYPEMSKEMFKLYIPGINSKVTELLLKADRTYSQMTDGLRDLWINVLSKLASKNDGSNYDLNEEINNISKVHTTYKSDKWYNPFKTWFTIKYDMRRLQKARNEITFNVGKDYNLLEDQKNFLLIHPELVLILDKQNYNGYLITPELVLMYCDVVEGRWNISACAKLDPKLQSMYQKGNNLWEVIDKLFPIMGEKTFDVISLLEPLALSLIQTHDPVKQLRGAFLNHVLSEMELIFESRESIKEFLSVDYIDKILDIFNKSTIDEIAEIFSFFRTFGHPPLEASIAAEKVRKYMYIGKQLKFDTINKCHAIFCTIIINGYRERHGGQWPPVTLPDHAHEFIINAYGSNSAISYENAVDYYQSFIGIKFNKFIEPQLDEDLTIYMKDKALSPKKSNWDTVYPASNLLYRTNASNESRRLVEVFIADSKFDPHQILDYVESGDWLDDPEFNISYSLKEKEIKQEGRLFAKMTYKMRATQVLSETLLANNIGKFFQENGMVKGEIELLKRLTTISISGVPRYNEVYNNSKSHTDDLKTYNKISNLNLSSNQKSKKFEFKSTDIYNDGYETVSCFLTTDLKKYCLNWRYESTALFGETCNQIFGLNKLFNWLHPRLEGSTIYVGDPYCPPSDKEHISLEDHPDSGFYVHNPRGGIEGFCQKLWTLISISAIHLAAVRIGVRVTAMVQGDNQAIAVTTRVPNNYDYRVKKEIVYKDVVRFFDSLREVMDDLGHELKLNETIISSKMFIYSKRIYYDGRILPQALKALSRCVFWSETVIDETRSASSNLATSFAKAIENGYSPVLGYACSIFKNIQQLYIALGMNINPTITQNIRDQYFRNPNWMQYASLIPASVGGFNYMAMSRCFVRNIGDPSVAALADIKRFIKANLLDRSVLYRIMNQEPGESSFLDWASDPYSCNLPQSQNITTMIKNITARNVLQDSPNPLLSGLFTNTMIEEDEELAEFLMDRKVILPRVAHDILDNSLTGIRNAIAGMLDTTKSLIRVGINRGGLTYSLLRKISNYDLVQYETLSRTLRLIVSDKIKYEDMCSVDLAIALRQKMWIHLSGGRMISGLETPDPLELLSGVVITGSEHCKICYSSDGTNPYTWMYLPGNIKIGSAETGISSLRVPYFGSVTDERSEAQLGYIKNLSKPAKAAIRIAMIYTWAFGNDEISWMEASQIAQTRANFTLDSLKILTPVATSTNLSHRLKDTATQMKFSSTSLIRVSRFITMSNDNMSIKEANETKDTNLIYQQIMLTGLSVFEYLFRLKETTGHNPIVMHLHIEDECCIKESFNDEHINPESTLELIRYPESNEFIYDKDPLKDVDLSKLMVIKDHSYTIDMNYWDDTDIIHAISICTAITIADTMSQLDRDNLKEIIVIANDDDINSLITEFLTLDILVFLKTFGGLLVNQFAYTLYSLKIEGRDLIWDYIMRTLRDTSHSILKVLSNALSHPKVFKRFWDCGVLNPIYGPNTASQDQIKLALSICEYSLDLFMREWLNGVSLEIYICDSDMEVANDRKQAFISRHLSFVCCLAEIASFGPNLLNLTYLERLDLLKQYLELNIKEDPTLKYVQISGLLIKSFPSTVTYVRKTAIKYLRIRGISPPEVIDDWDPVEDENMLDNIVKTINDNCNKDNKGNKINNFWGLALKNYQVLKIRSITSDSDDNDRLDANTSGLTLPQGGNYLSHQLRLFGINSTSCLKALELSQILMKEVNKDKDRLFLGEGAGAMLACYDATLGPAVNYYNSGLNITDVIGQRELKIFPSEVSLVGKKLGNVTQILNRVKVLFNGNPNSTWIGNMECESLIWSELNDKSIGLVHCDMEGAIGKSEETVLHEHYSVIRITYLIGDDDVVLVSKIIPTITPNWSRILYLYKLYWKDVSIISLKTSNPASTELYLISKDAYCTIMEPSEIVLSKLKRLSLLEENNLLKWIILSKKRNNEWLHHEIKEGERDYGIMRPYHMALQIFGFQINLNHLAKEFLSTPDLTNINNIIQSFQRTIKDVLFEWINITHDDKRHKLGGRYNIFPLKNKGKLRLLSRRLVLSWISLSLSTRLLTGRFPDEKFEHRAQTGYVSLADTDLESLKLLSKNIIKNYRECIGSISYWFLTKEVKILMKLIGGAKLLGIPRQYKEPEDQLLENYNQHDEFDID

SEQ ID NO: 46 - protein, 46 aa, Human parainfluenza virus 3
IIIILIMIIILFIINITIITIAIKYYRIQKRNRVDQNDKPYVLTNK

SEQ ID NO: 47 - protein, 515 aa, Bovine parainfluenza virus 3
MLSLFDTFSARRQENITKSAGGAVIPGQKNTVSIFALGPSITDDNDKMTLALLFLSHSLDNEKQHAQRAGFLVSLLSMAYANPELYLTSNGSNADVKYVIYMIEKDPGRQKYGGFVVKTREMVYEKTTDWMFGSDLEYDQDNMLQNGRSTSTIEDLVHTFGYPSCLGALIIQVWIILVKAITSISGLRKGFFTRLEAFRQDGTVKSSLVLSGDAVEQIGSIMRSQQSLVTLMVETLITMNTGRNDLTTIEKNIQIVGNYIRDAGLASFFNTIRYGIETRMAALTLSTLRPDINRLKALIELYLSKGPRAPFICILRDPVHGEFAPGNYPALWSYAMGVAVVQNKAMQQYVTGRSYLDIEMFQLGQAVARDAESQMSSILEDELGVTQEAKQSLKKHMKNISSSDTTFHKPTGGSAIEMAIDEEAGQPESRGDQDQGDEPRSSIVPYAWADETGNDNQTESTTEIDSIKTEQRNIRDRLNKRLNEKRKQSDPRSTDITNNTNQTEIDDLFSAFGSN

SEQ ID NO: 48 - protein, 596 aa, Bovine parainfluenza virus 3
MEDNVQNNQIMDSWEEGSGDKSSDISSALDIIEFILSTDSQENTADSNEINTGTTRLSTTIYQPESKTTETSKENSGPANKNRQFGASHERATETKDRNVNQETVQGGYRRGSSPDSRTETMVTRRISRSSPDPNNGTQIQEDIDYNEVGEMDKDSTKREMRQFKDVPVKVSGSDAIPPTKQDGDGDDGRGLESISTFDSGYTSIVTAATLDDEEELLMKNNRPRKYQSTPQNSDKGIKKGVGRPKDTDKQSSILDYELNFKGSKKSQKILKASTNTGEPTRPQNGSQGKRITSWNILNSESGNRTESTNQTHQTSTSGQNHTMGPSRTTSEPRIKTQKTDGKEREDTEESTRFTERAITLLQNLGVIQSAAKLDLYQDKRVVCVANVLNNADTASKIDFLAGLMIGVSMDHDTKLNQIQNEILSLKTDLKKMDESHRRLIENQKEQLSLITSLISNLKIMTERGGKKDQPEPSGRTSMIKTKAKEEKIKKVRFDPLMETQGIEKNIPDLYRSIEKTPENDTQIKSEINRLNDESNATRLVPRRISSTMRSLIIIINNSNLSSKAKQSYINELKLCKSDEEVSELMDMFNEDVSSQ

SEQ ID NO: 49 - protein, 351 aa, Bovine parainfluenza virus 3
MSITNSTIYTFPESSFSENGNIEPLPLKVNEQRKAIPHIRVVKIGDPPKHGSRYLDVFLLGFFEMERSKDRYGSISDLDDDPSYKVCGSGSLPLGLARYTGNDQELLQAATKLDIEVRRTVKATEMIVYTVQNIKPELYPWSSRLRKGMLFDANKVALAPQCLPLDRGIKFRVIFVNCTAIGSITLFKIPKSMALLSLPNTISINLQVHIKTGVQTDSKGVVQILDEKGEKSLNFMVHLGLIKRKMGRMYSVEYCKQKIEKMRLLFSLGLVGGISFHVNATGSISKTLASQLAFKREICYPLMDLNPHLNSVIWASSVEITRVDAVLQPSLPGEFRYYPNIIAKGVGKIRQ

SEQ ID NO: 50 - protein, 540 aa, Bovine parainfluenza virus 3
MTITTTIIAILLIPPSFCQIDITKLQRVGVLVNNPKGMKISQNFETRYLILSLIPKIENSHSCGDQQINQYKKLLDRLIIPLYDGLKLQKDVIVVSHETHNNTNLRTKRFFGEIIGTIAIGIATSAQITAAVALVEAKQAKSDIEKLKEAIRDTNKAVQSIQSSVGNLIVAVKSVQDYVNNEIIPSITRLGCEAAGLQLGIALTQHYSELTNIFGDNIGTLKEKGIKLQGIASLYHTNITEIFTTSTVDQYDIYDLLFTESIKMRVIDVDLSDYSITLQVRLPLLTKLSNTQIYKVDSISYNIQGKEWYIPLPNHIMTKGAFLGGADIKECIEAFSSYICPSDPGYILNHEIENCLSGNITQCPKTVVTSDVVPRYAFVNGGLIANCITTTCTCNGIDNRINQSPDQGIKIITHKECQVIGINGMLFNTNREGTLATYTFDDIILNNSVALNPIDISMELNKAKLELEESKEWIKKSNQKLDSVGSWYQSSATITIIIVMIIILVIINITIIVVIIKFHRIQGKDQNDKNSEPYILTNRQ

SEQ ID NO: 51 - protein, 572 aa, Bovine parainfluenza virus 3
MEYWKHTNSINNTNNETETARGKHSSKVTNIIMYTFWTITLTILSVIFIMILTNLIQENNHNKLMLQEIRKEFAAIDTKIQRTSDDIGTSIQSGINTRLLTIQSHVQNYIPLSLTQQMSDLRKFINDLTNKREHQEVPIQRMTHDRGIEPLNPNKFWRCTSGNPSLTSSPKIRLIPGPGLLATSTTVNGCIRIPSLVINHLIYAYTSNLITQGCQDIGKSYQVLQIGIITINSDLVPDLNPRVTHTFNIDDNRRSCSLALLNTDVYQLCSTPKVDERSDYASTGIEDIVLDIVTNNGLIITTRFTNNNITFDKPYAALYPSVGPGIYYKDKVIFLGYGGLEHEENGDVICNTTGCPGKTQRDCNQASYSPWFSNRRMVNSIIVVDKGIDATFSLRVWTIPMSQNYWGSEGRLLLLGDRIYIYTRSTSWHSKLQLGVIDISDYTNIRINWTWHNVLSRPGNDECPWGHSCPDGCITGVYTDAYPLNPSGSVVSSVILDSQKSRENPIITYSTATNRINELAIYNRTLPAAYTTTNCITHYDKGYCFHIVEINHRSLNTFQPMLFKTEVPKNCS

SEQ ID NO: 52 - protein, 2233 aa, Bovine parainfluenza virus 3
MDTESHSGTTSDILYPECHLNSPIVKGKIAQLHTIMSLPQPYDMDDDSILIITRQKIKLNKLDKRQRSIRKLRSVLMERVSDLGKYTFIRYPEMSSEMFQLCIPGINNKINELLSKASKTYNQMTDGLRDLWVTILSKLASKNDGSNYDINEDISNISNVHMTYQSDKWYNPFKTWFTIKYDMRRLQKAKNEITFNRHKDYNLLEDQKNILLIHPELVLILDKQNYNGYIMTPELVLMYCDVVEGRWNISSCAKLDPKLQSMYYKGNNLWEIIDGLFSTLGERTFDIISLLEPLALSLIQTYDPVKQLRGAFLNHVLSEMELIFAAECTTEEIPNVDYIDKILDVFKESTIDEIAEIFSFFRTFGHPPLEASIAAEKVRKYMYTEKCLKFDTINKCHAIFCTIIINGYRERHGGQWPPVTLPVHAHEFIINAYGSNSAISYENAVDYYKSFIGIKFDKFIEPQLDEDLTIYMKDKALSPKKSNWDTVYPASNLLYRTNVSHDSRRLVEVFIADSKFDPHQVLDYVESGYWLDDPEFNISYSLKEKEIKQEGRLFAKMTYKMRATQVLSETLLANNIGKFFQENGMVKGEIELLKRLTTISMSGVPRYNEVYNNSKSHTEELQAYNAISSSNLSSNQKSKKFEFKSTDIYNDGYETVSCFLTTDLKKYCLNWRYESTALFGDTCNQIFGLKELFNWLHPRLEKSTIYVGDPYCPPSDIEHLPLDDHPDSGFYVHNPKGGIEGFCQKLWTLISISAIHLAAVKIGVRVTAMVQGDNQAIAVTTRVPNNYDYKVKKEIVYKDVVRFFDSLREVMDDLGHELKLNETIISSKMFIYSKRIYYDGRILPQALKALSRCVFWSETIIDETRSASSNLATSFAKAIENGYSPVLGYVCSIFKNIQQLYIALGMNINPTITQNIKDQYFRNIHWMQYASLIPASVGGFNYMAMSRCFVRNIGDPTVAALADIKRFIKANLLDRGVLYRIMNQEPGESSFLDWASDPYSCNLPQSQNITTMIKNITARNVLQDSPNPLLSGLFTSTMIEEDEELAEFLMDRRIILPRVAHDILDNSLTGIRNAIAGMLDTTKSLIRVGISRGGLTYNLLRKISNYDLVQYETLSKTLRLIVSDKIKYEDMCSVDLAISLRQKMWMHLSGGRMINGLETPDPLELLSGVIITGSEHCRICYSTEGESPYTWMYLPGNLNIGSAETGIASLRVPYFGSVTDERSEAQLGYIKNLSKPAKAAIRIAMIYTWAFGNDEISWMEASQIAQTRANFTLDSLKILTPVTTSTNLSHRLKDTATQMKFSSTSLIRVSRFITISNDNMSIKEANETKDTNLIYQQVMLTGLSVFEYLFRLEESTGHNPMVMHLHIEDGCCIKESYNDEHINPESTLELIKYPESNEFIYDKDPLKDIDLSKLMVIRDHSYTIDMNYWDDTDIVHAISICTAVTIADTMSQLDRDNLKELVVIANDDDINSLITEFLTLDILVFLKTFGGLLVNQFAYTLYGLKIEGRDPIWDYIMRTLKDTSHSVLKVLSNALSHPKVFKRFWDCGVLNPIYGPNTASQDQVKLALSICEYSLDLFMREWLNGASLEIYICDSDMEIANDRRQAFLSRHLAFVCCLAEIASFGPNLLNLTYLERLDELKQYLDLNIKEDPTLKYVQVSGLLIKSFPSTVTYVRKTAIKYLRIRGINPPETIEDWDPIEDENILDNIVKTVNDNCSDNQKRNKSSYFWGLALKNYQVVKIRSITSDSEVNEASNVTTHGMTLPQGGSYLSHQLRLFGVNSTSCLKALELSQILMREVKKDKDRLFLGEGAGAMLACYDATLGPAINYYNSGLNITDVIGQRELKIFPSEVSLVGKKLGNVTQILNRVRVLFNGNPNSTWIGNMECESLIWSELNDKSIGLVHCDMEGAIGKSEETVLHEHYSIIRITYLIGDDDVVLVSKIIPTITPNWSKILYLYKLYWKDVSVVSLKTSNPASTELYLISKDAYCTVMEPSNLVLSKLKRISSIEENNLLKWIILSKRKNNEWLQHEIKEGERDYGIMRPYHTALQIFGFQINLNHLAREFLSTPDLTNINNIIQSFTRTIKDVMFEWVNITHDNKRHKLGGRYNLFPLKNKGKLRLLSRRLVLSWISLSLSTRLLTGRFPDEKFENRAQTGYVSLADIDLESLKLLSRNIVKNYKEHIGLISYWFLTKEVKILMKLIGGVKLLGIPKQYKELEDRSSQGYEYDNEFDID

SEQ ID NO: 53 - protein, 47 aa, Bovine parainfluenza virus 3
ITIIIVMIIILVIINITIIVVIIKFHRIQGKDQNDKNSEPYILTNRQ

SEQ ID NO: 54 - DNA, 10 bp, Human parainfluenza virus 1
agggttaaag

SEQ ID NO: 55 - DNA, 12 bp, Human parainfluenza virus 1
aagtaagaaaaa

SEQ ID NO: 56 - DNA, 10 bp, Human parainfluenza virus 1
agggtgaatg

SEQ ID NO: 57 - DNA, 12 bp, Human parainfluenza virus 1
aattaagaaaaa

SEQ ID NO: 58 - DNA, 10 bp, Human parainfluenza virus 1
agggtcaaag

SEQ ID NO: 59 - DNA, 12 bp, Human parainfluenza virus 1
aaataagaaaaa

SEQ ID NO: 60 - DNA, 10 bp, Human parainfluenza virus 1
agggacaaag

SEQ ID NO: 61 - DNA, 10 bp, Human parainfluenza virus 1
agggttaaag

SEQ ID NO: 62 - DNA, 12 bp, Human parainfluenza virus 1
gaataagaaaaa

SEQ ID NO: 63 - DNA, 10 bp, Human parainfluenza virus 1
agggttaatg

SEQ ID NO: 64 - DNA, 12 bp, Human parainfluenza virus 1
tagtaagaaaaa

SEQ ID NO: 65 - DNA, 14 bp, Human parainfluenza virus 2
agattccggtgccg

SEQ ID NO: 66 - DNA, 14 bp, Human parainfluenza virus 2
aatttaagaaaaaa

SEQ ID NO: 67 - DNA, 17 bp, Human parainfluenza virus 2
aggcccggacgggttag

SEQ ID NO: 68 - DNA, 14 bp, Human parainfluenza virus 2
aatttaataaaaaa

SEQ ID NO: 69 - DNA, 12 bp, Human parainfluenza virus 2
aggtccgaaagc

SEQ ID NO: 70 - DNA, 15 bp, Human parainfluenza virus 2
aatctaacaaaaaaa

SEQ ID NO: 71 - DNA, 12 bp, Human parainfluenza virus 2
aggccaaattat

SEQ ID NO: 72 - DNA, 14 bp, Human parainfluenza virus 2
aatttaagaaaaaa

SEQ ID NO: 73 - DNA, 12 bp, Human parainfluenza virus 2
aagcacgaaccc

SEQ ID NO: 74 - DNA, 14 bp, Human parainfluenza virus 2
tatttaagaaaaaa

SEQ ID NO: 75 - DNA, 8 bp, Human parainfluenza virus 2
aggccaga

SEQ ID NO: 76 - DNA, 13 bp, Human parainfluenza virus 2
tatttaagaaaaa

SEQ ID NO: 77 - DNA, 12 bp, Human parainfluenza virus 3
aggattaaagac

SEQ ID NO: 78 - DNA, 12 bp, Human parainfluenza virus 3
aaataagaaaaa

SEQ ID NO: 79 - DNA, 10 bp, Human parainfluenza virus 3
aggattaaag

SEQ ID NO: 80 - DNA, 12 bp, Human parainfluenza virus 3
aaataagaaaaa

SEQ ID NO: 81 - DNA, 10 bp, Human parainfluenza virus 3
aggattaaag

SEQ ID NO: 82 - DNA, 20 bp, Human parainfluenza virus 3
aaataaaggataatcaaaaa

SEQ ID NO: 83 - DNA, 10 bp, Human parainfluenza virus 3
aggacaaaag

SEQ ID NO: 84 - DNA, 12 bp, Human parainfluenza virus 3
aattataaaaaa

SEQ ID NO: 85 - DNA, 10 bp, Human parainfluenza virus 3
aggagtaaag

SEQ ID NO: 86 - DNA, 12 bp, Human parainfluenza virus 3
aaatataaaaaa

SEQ ID NO: 87 - DNA, 10 bp, Human parainfluenza virus 3
aggagcaaag

SEQ ID NO: 88 - DNA, 13 bp, Human parainfluenza virus 3
aaagtaagaaaaa

SEQ ID NO: 89 - protein, 12 aa, Bovine parainfluenza virus 3
AGGATTAAAGAA

SEQ ID NO: 90 - protein, 13 aa, Bovine parainfluenza virus 3
CAAGTAAGAAAAA

SEQ ID NO: 91 - protein, 12 aa, Bovine parainfluenza virus 3
AGGATTAATGGA

SEQ ID NO: 92 - protein, 13 aa, Bovine parainfluenza virus 3
TGATTAAGAAAAA

SEQ ID NO: 93 - protein, 12 aa, Bovine parainfluenza virus 3
AGGATGAAAGGA

SEQ ID NO: 94 - protein, 13 aa, Bovine parainfluenza virus 3
GAAAAATCAAAAA

SEQ ID NO: 95 - protein, 12 aa, Bovine parainfluenza virus 3
AGGATCAAAGGG

SEQ ID NO: 96 - protein, 14 aa, Bovine parainfluenza virus 3
AAAAGTACAAAAAA

SEQ ID NO: 97 - protein, 12 aa, Bovine parainfluenza virus 3
AGGAACAAAGTT

SEQ ID NO: 98 - protein, 14 aa, Bovine parainfluenza virus 3
GAAATAATAAAAAA

SEQ ID NO: 99 - protein, 12 aa, Bovine parainfluenza virus 3
AGGAGAAAAGTG

SEQ ID NO: 100 - protein, 13 aa, Bovine parainfluenza virus 3
AAAGTAAGAAAAA

SEQ ID NO: 101 - protein, 572 aa, Human parainfluenza virus 3
MEYWKHTNHGKDAGNELETSMATHGNKLTNKIIYILWTIILVLLSIVFIIVLINSIKSEKAHESLLQDINNEFMEITEKIQMASDNTNDLIQSGVNTRLLTIQSHVQNYIPISLTQQMSDLRKFISEITIRNDNQEVLPQRITHDVGIKPLNPDDFWRCTSGLPSLMKTPKIRLMPGPGLLAMPTTVDGCVRTPSLVINDLIYAYTSNLITRGCQDIGKSYQVLQIGIITVNSDLVPDLNPRISHTFNINDNRKSCSLALLNIDVYQLCSTPKVDERSDYASSGIEDIVLDIVNYDGSISTTRFKNNNISFDQPYAALYPSVGPGIYYKGKIIFLGYGGLEHPINENVICNTTGCPGKTQRDCNQASHSTWFSDRRMVNSIIVVDKGLNSIPKLKVWTISMRQNYWGSEGRLLLLGNKIYIYTRSTSWHSKLQLGIIDITDYSDIRIKWTWHNVLSRPGNNECPWGHSCPDGCITGVYTDAYPLNPTGSIVSSVILDSQKSRVNPVITYSTATERVNELAILNRTLSAGYTTTSCITHYNKGYCFHIVEINHKSLNTFQPMLFKTEIPKSCS

SEQ ID NO: 102 - protein, 1719 aa, Human parainfluenza virus 3
ATGGAATACTGGAAGCATACCAATCACGGAAAGGATGCTGGTAATGAGCTGGAGACGTCTATGGCTACTCATGGCAACAAGCTCACTAATAAGATAATATACATATTATGGACAATAATCCTGGTGTTATTATCAATAGTCTTCATCATAGTGCTAATTAATTCCATCAAAAGTGAAAAGGCCCACGAATCATTGCTGCAAGACATAAATAATGAGTTTATGGAAATTACAGAAAAGATCCAAATGGCATCGGATAATACCAATGATCTAATACAGTCAGGAGTGAATACAAGGCTTCTTACAATTCAGAGTCATGTCCAGAATTACATACCAATATCATTGACACAACAGATGTCAGATCTTAGGAAATTCATTAGTGAAATTACAATTAGAAATGATAATCAAGAAGTGCTGCCACAAAGAATAACACATGATGTAGGTATAAAACCTTTAAATCCAGATGATTTTTGGAGATGCACGTCTGGTCTTCCATCTTTAATGAAAACTCCAAAAATAAGGTTAATGCCAGGGCCGGGATTATTAGCTATGCCAACGACTGTTGATGGCTGTGTTAGAACTCCGTCTTTAGTTATAAATGATCTGATTTATGCTTATACCTCAAATCTAATTACTCGAGGTTGTCAGGATATAGGAAAATCATATCAAGTCTTACAGATAGGGATAATAACTGTAAACTCAGACTTGGTACCTGACTTAAATCCTAGGATCTCTCATACCTTTAACATAAATGACAATAGGAAGTCATGTTCTCTAGCACTCCTAAATATAGATGTATATCAACTGTGTTCAACTCCCAAAGTTGATGAAAGATCAGATTATGCATCATCAGGCATAGAAGATATTGTACTTGATATTGTCAATTATGATGGTTCAATCTCAACAACAAGATTTAAGAATAATAACATAAGCTTTGATCAACCATATGCTGCACTATACCCATCTGTTGGACCAGGGATATACTACAAAGGCAAAATAATATTTCTCGGGTATGGAGGTCTTGAACATCCAATAAATGAGAATGTAATCTGCAACACAACTGGGTGCCCCGGGAAAACACAGAGAGACTGTAATCAAGCATCTCATAGTACTTGGTTTTCAGATAGGAGGATGGTCAACTCCATCATTGTTGTTGACAAAGGCTTAAACTCAATTCCAAAATTGAAAGTATGGACGATATCTATGCGACAAAATTACTGGGGGTCAGAAGGAAGGTTACTTCTACTAGGTAACAAGATCTATATATATACAAGATCTACAAGTTGGCATAGCAAGTTACAATTAGGAATAATTGATATTACTGATTACAGTGATATAAGGATAAAATGGACATGGCATAATGTGCTATCAAGACCAGGAAACAATGAATGTCCATGGGGACATTCATGTCCAGATGGATGTATAACAGGAGTATATACTGATGCATATCCACTCAATCCCACAGGGAGCATTGTGTCATCTGTCATATTAGACTCACAAAAATCGAGAGTGAACCCAGTCATAACTTACTCAACAGCAACCGAAAGAGTAAACGAGCTGGCCATCCTAAACAGAACACTCTCAGCTGGATATACAACAACAAGCTGCATTACACACTATAACAAAGGATATTGTTTTCATATAGTAGAAATAAATCATAAAAGCTTAAACACATTTCAACCCATGTTGTTCAAAACAGAGATTCCAAAAAGCTGCAGTTAA

SEQ ID NO: 103 - protein, 65 aa, Sendai virus
VITIIVVMVVILVVIIVIIIVLYRLRRSMLMGNPDDRIPRDTYTLEPKIRHMYTNGGFDAMAEKR

SEQ ID NO: 104 - protein, 49 aa, Newcastle disease virus
IVLTIISLVFGILSLILACYLMYKQKAQQKTLLWLGNNTLDQMRATTKM

SEQ ID NO: 105 - protein, 594 aa, Artificial sequence
  Recombinant RSV F
MELLILKANAITTILTAVTFCFASGQNITEEFYQSTCSAVSKGYLSALRTGWYTSVITIELSNIKENKCNGTDAKVKLIKQELDKYKNAVTELQLLMQSTPATNNRARRELPRFMNYTLNNAKKTNVTLSKKRKRRFLGFLLGVGSAIASGVAVSKVLHLEGEVNKIKSALLSTNKAVVSLSNGVSVLTSKVLDLKNYIDKQLLPIVNKQSCSISNIETVIEFQQKNNRLLEITREFSVNAGVTTPVSTYMLTNSELLSLINDMPITNDQKKLMSNNVQIVRQQSYSIMSIIKEEVLAYVVQLPLYGVIDTPCWKLHTSPLCTTNTKEGSNICLTRTDRGWYCDNAGSVSFFPQAETCKVQSNRVFCDTMNSLTLPSEVNLCNVDIFNPKYDCKIMTSKTDVSSSVITSLGAIVSCYGKTKCTASNKNRGIIKTFSNGCDYVSNKGVDTVSVGNTLYYVNKQEGKSLYVKGEPIINFYDPLVFPSDEFDASISQVNEKINQSLAFIRKSDELLHNVNAGKSTTNIMITTIIIVIIVILLSLIAVGLLLYCLYRLRRSMLMGNPDDRIPRDTYTLEPKIRHMYTNGGFDAMAEKR

SEQ ID NO: 106 - protein, 594 aa, Artificial sequence
  Recombinant RSV F
MELLILKANAITTILTAVTFCFASGQNITEEFYQSTCSAVSKGYLSALRTGWYTSVITIELSNIKENKCNGTDAKVKLIKQELDKYKNAVTELQLLMQSTPATNNRARRELPRFMNYTLNNAKKTNVTLSKKRKRRFLGFLLGVGSAIASGVAVSKVLHLEGEVNKIKSALLSTNKAVVSLSNGVSVLTSKVLDLKNYIDKQLLPIVNKQSCSISNIETVIEFQQKNNRLLEITREFSVNAGVTTPVSTYMLTNSELLSLINDMPITNDQKKLMSNNVQIVRQQSYSIMSIIKEEVLAYVVQLPLYGVIDTPCWKLHTSPLCTTNTKEGSNICLTRTDRGWYCDNAGSVSFFPQAETCKVQSNRVFCDTMNSLTLPSEVNLCNVDIFNPKYDCKIMTSKTDVSSSVITSLGAIVSCYGKTKCTASNKNRGIIKTFSNGCDYVSNKGVDTVSVGNTLYYVNKQEGKSLYVKGEPIINFYDPLVFPSDEFDASISQVNEKINQSLAFIRKSDELLHNVNAGKSTTNIMITTVITIIVVMVVILVVIIVIIIVLYRLRRSMLMGNPDDRIPRDTYTLEPKIRHMYTNGGFDAMAEKR

SEQ ID NO: 107 - protein, 594 aa, Artificial sequence
  Recombinant RSV F
MELLILKANAITTILTAVTFCFASGQNITEEFYQSTCSAVSKGYLSALRTGWYTSVITIELSNIKENKCNGTDAKVKLIKQELDKYKNAVTELQLLMQSTPATNNRARRELPRFMNYTLNNAKKTNVTLSKKRKRRFLGFLLGVGSAIASGVAVCKVLHLEGEVNKIKSALLSTNKAVVSLSNGVSVLTFKVLDLKNYIDKQLLPILNKQSCSISNIETVIEFQQKNNRLLEITREFSVNAGVTTPVSTYMLTNSELLSLINDMPITNDQKKLMSNNVQIVRQQSYSIMCIIKEEVLAYVVQLPLYGVIDTPCWKLHTSPLCTTNTKEGSNICLTRTDRGWYCDNAGSVSFFPQAETCKVQSNRVFCDTMNSLTLPSEVNLCNVDIFNPKYDCKIMTSKTDVSSSVITSLGAIVSCYGKTKCTASNKNRGIIKTFSNGCDYVSNKGVDTVSVGNTLYYVNKQEGKSLYVKGEPIINFYDPLVFPSDEFDASISQVNEKINQSLAFIRKSDELLHNVNAGKSTTNIMITTIIIVIIVILLSLIAVGLLLYCLYRLRRSMLMGNPDDRIPRDTYTLEPKIRHMYTNGGFDAMAEKR

SEQ ID NO: 108 - protein, 594 aa, Artificial sequence
  Recombinant RSV F
MELLILKANAITTILTAVTFCFASGQNITEEFYQSTCSAVSKGYLSALRTGWYTSVITIELSNIKENKCNGTDAKVKLIKQELDKYKNAVTELQLLMQSTPATNNRARRELPRFMNYTLNNAKKTNVTLSKKRKRRFLGFLLGVGSAIASGVAVCKVLHLEGEVNKIKSALLSTNKAVVSLSNGVSVLTFKVLDLKNYIDKQLLPILNKQSCSISNIETVIEFQQKNNRLLEITREFSVNAGVTTPVSTYMLTNSELLSLINDMPITNDQKKLMSNNVQIVRQQSYSIMCIIKEEVLAYVVQLPLYGVIDTPCWKLHTSPLCTTNTKEGSNICLTRTDRGWYCDNAGSVSFFPQAETCKVQSNRVFCDTMNSLTLPSEVNLCNVDIFNPKYDCKIMTSKTDVSSSVITSLGAIVSCYGKTKCTASNKNRGIIKTFSNGCDYVSNKGVDTVSVGNTLYYVNKQEGKSLYVKGEPIINFYDPLVFPSDEFDASISQVNEKINQSLAFIRKSDELLHNVNAGKSTTNIMITTVITIIVVMVVILVVIIVIIIVLYRLRRSMLMGNPDDRIPRDTYTLEPKIRHMYTNGGFDAMAEKR

SEQ ID NO: 109 - protein, 578 aa, Artificial sequence
  Recombinant RSV F
MELLILKANAITTILTAVTFCFASGQNITEEFYQSTCSAVSKGYLSALRTGWYTSVITIELSNIKENKCNGTDAKVKLIKQELDKYKNAVTELQLLMQSTPATNNRARRELPRFMNYTLNNAKKTNVTLSKKRKRRFLGFLLGVGSAIASGVAVSKVLHLEGEVNKIKSALLSTNKAVVSLSNGVSVLTSKVLDLKNYIDKQLLPIVNKQSCSISNIETVIEFQQKNNRLLEITREFSVNAGVTTPVSTYMLTNSELLSLINDMPITNDQKKLMSNNVQIVRQQSYSIMSIIKEEVLAYVVQLPLYGVIDTPCWKLHTSPLCTTNTKEGSNICLTRTDRGWYCDNAGSVSFFPQAETCKVQSNRVFCDTMNSLTLPSEVNLCNVDIFNPKYDCKIMTSKTDVSSSVITSLGAIVSCYGKTKCTASNKNRGIIKTFSNGCDYVSNKGVDTVSVGNTLYYVNKQEGKSLYVKGEPIINFYDPLVFPSDEFDASISQVNEKINQSLAFIRKSDELLHNVNAGKSTTNIMITTIIIVIIVILLSLIAVGLLLYCMYKQKAQQKTLLWLGNNTLDQMRATTKM

SEQ ID NO: 110 - protein, 578 aa, Artificial sequence
  Recombinant RSV F
MELLILKANAITTILTAVTFCFASGQNITEEFYQSTCSAVSKGYLSALRTGWYTSVITIELSNIKENKCNGTDAKVKLIKQELDKYKNAVTELQLLMQSTPATNNRARRELPRFMNYTLNNAKKTNVTLSKKRKRRFLGFLLGVGSAIASGVAVSKVLHLEGEVNKIKSALLSTNKAVVSLSNGVSVLTSKVLDLKNYIDKQLLPIVNKQSCSISNIETVIEFQQKNNRLLEITREFSVNAGVTTPVSTYMLTNSELLSLINDMPITNDQKKLMSNNVQIVRQQSYSIMSIIKEEVLAYVVQLPLYGVIDTPCWKLHTSPLCTTNTKEGSNICLTRTDRGWYCDNAGSVSFFPQAETCKVQSNRVFCDTMNSLTLPSEVNLCNVDIFNPKYDCKIMTSKTDVSSSVITSLGAIVSCYGKTKCTASNKNRGIIKTFSNGCDYVSNKGVDTVSVGNTLYYVNKQEGKSLYVKGEPIINFYDPLVFPSDEFDASISQVNEKINQSLAFIRKSDELLHNVNAGKSTTNIMITTIVLTIISLVFGILSLILACYLMYKQKAQQKTLLWLGNNTLDQMRATTKM

SEQ ID NO: 111 - DNA, 49 bp, Artificial sequence
  Oligonucleotide primer
gcggccgccgtacgctatcagttggagaaggcgatattgttgatgccgg

SEQ ID NO: 112 - protein, 578 aa, Artificial sequence
  Recombinant RSV F
MELLILKANAITTILTAVTFCFASGQNITEEFYQSTCSAVSKGYLSALRTGWYTSVITIELSNIKENKCNGTDAKVKLIKQELDKYKNAVTELQLLMQSTPATNNRARRELPRFMNYTLNNAKKTNVTLSKKRKRRFLGFLLGVGSAIASGVAVCKVLHLEGEVNKIKSALLSTNKAVVSLSNGVSVLTFKVLDLKNYIDKQLLPILNKQSCSISNIETVIEFQQKNNRLLEITREFSVNAGVTTPVSTYMLTNSELLSLINDMPITNDQKKLMSNNVQIVRQQSYSIMCIIKEEVLAYVVQLPLYGVIDTPCWKLHTSPLCTTNTKEGSNICLTRTDRGWYCDNAGSVSFFPQAETCKVQSNRVFCDTMNSLTLPSEVNLCNVDIFNPKYDCKIMTSKTDVSSSVITSLGAIVSCYGKTKCTASNKNRGIIKTFSNGCDYVSNKGVDTVSVGNTLYYVNKQEGKSLYVKGEPIINFYDPLVFPSDEFDASISQVNEKINQSLAFIRKSDELLHNVNAGKSTTNIMITTIIIVIIVILLSLIAVGLLLYCMYKQKAQQKTLLWLGNNTLDQMRATTKM

SEQ ID NO: 113 - protein, 594 aa, Artificial sequence; identical to SEQ ID NO: 108
  Recombinant RSV F

SEQ ID NO: 114 - protein, 199 aa, Human parainfluenza virus 3
MLKTIKSWILGKRNQEINQLISPRPSTSLNSYSAPTPKKTYRKTTQSTQEPSNSVPPSVNQKSNQQKQVRKIVDQLTKIDSPGHHTNVQQKQKIEILIRKLYREDLGEEAAQIVELRLWSLEESPEASQILKMEPKTRRILISMKLERWIRTLLRGKCDNLQMFQARYQEVMTYLQQNKVETVIMEEAWNLSVHLIQDQ

SEQ ID NO: 115 - protein, 201 aa, Bovine parainfluenza virus 3
MFKTIKSWILGKRDQEINHLTSHRPSTSLNSYSAPTPKRTRQTAMKSTQEPQDLARQSTNLNPKQQKQARKIVDQLTKIDSLGHHTNVPQRQKIEMLIRRLYREDIGEEAAQIVELRLWSLEESPEAAQILTMEPKSRKILITMKLERWIRTLLRGKCDNLKMFQSRYQEVMPFLQQNKMETVMMEEAWNLSVHLIQDIPV

SEQ ID NO: 116 - protein, 412 aa, Bovine parainfluenza virus 3
MEDNVQNNQIMDSWEEGSGDKSSDISSALDIIEFILSTDSQENTADSNEINTGTTRLSTTIYQPESKTTETSKENSGPANKNRQFGASHERATETKDRNVNQETVQGGYRRGSSPDSRTETMVTRRISRSSPDPNNGTQIQEDIDYNEVGEMDKDSTKREMRQFKDVPVKVSGSDAIPPTKQDGDGDDGRGLESISTFDSGYTSIVTAATLDDEEELLMKNNRPRKYQSTPQNSDKGIKKGGWKAKRHRQTIINIGLRTQLQRIEEEPENPQSQHEYRRTNKTTEWIPGEENHILEHPQQRERQSNRINKPNPSDINLGTEPHNGTKQNNLRTKDQDTKDGWKGKRGHRREHSIYRKGDYIITESWCNPICSKIRPIPRQESCVCGECPKQCRYCIKDRLPSRFDDRSVNGS

SEQ ID NO: 117 - DNA, 46 bp, human parainfluenza virus 2
ttaaaagaagttaagtaaaatttaaagaacacaatagagaaaacct

SEQ ID NO: 118 - DNA, 28 bp, human parainfluenza virus 2
ctaaacattcaataataaatcaaagttc

SEQ ID NO: 119 - DNA, 8 bp, human parainfluenza virus 2
cctaaaat

SEQ ID NO: 120 - DNA, 42 bp, human parainfluenza virus 2
taatctttatataatgtaacaatactactaagattataatat

SEQ ID NO: 121 - DNA, 34 bp, Artificial sequence
  Oligonucleotide primer
aagaagaccaagttgagccagaagaggtacgaag

SEQ ID NO: 122 - DNA, 34 bp, Artificial sequence
  Oligonucleotide primer
cttcgtacctcttctggctcaacttggtcttctt

SEQ ID NO: 123 - DNA, 51 bp, Artificial sequence
  Oligonucleotide primer
ccagctaacataggagggttcaacgcgatgtctacagctagatgttttgtc

SEQ ID NO: 124 - DNA, 51 bp, Artificial sequence
  Oligonucleotide primer
gacaaaacatctagctgtagacatcgcgttgaaccctcctatgttagctgg

SEQ ID NO: 125 - DNA, 12 bp, Human parainfluenza virus 1
aagtaagaaaaa

SEQ ID NO: 126 - DNA, 10 bp, Human parainfluenza virus 1
agggtgaatg

SEQ ID NO: 127 - DNA, 46 bp, Artificial sequence
  Oligonucleotide primer
acgcgtcccgggaacaatggaactgctgatcctgaaggccaacgcc

SEQ ID NO: 128 - DNA, 73 bp, Artificial sequence
  Oligonucleotide primer
acgcgtcgtacgcattcaccctaagtttttcttactttctatcagttggagaaggcgatattgttgatgccgg

SEQ ID NO: 129 - DNA, 48 bp, Artificial sequence
  Oligonucleotide primer
ggcgcgcccccgggaacaatggaactgctgatcctgaaggccaacgcc

SEQ ID NO: 130 - DNA, 79 bp, Artificial sequence
  Oligonucleotide primer
ggcgcgcccgtacgccattcaccctaagtttttcttacttgattctatcagttggagaaggcgatattgttgatgccgg

SEQ ID NO: 131 - DNA, 72 bp, Artificial sequence
  Oligonucleotide primer
gcggccgcccgggaagtaagaaaaacttagggtgaatgaacaatggaactgctgatcctgaaggccaacgcc

SEQ ID NO: 132 - protein, 31 aa, Artificial sequence
  linker and foldon domain
SAIGGYIPEAPRDGQAYVRKDGEWVLLSTFL

SEQ ID NO: 133 - protein, 586 aa, Artificial sequence
  Recombinant RSV F
MELLILKANAITTILTAVTFCFASGQNITEEFYQSTCSAVSKGYLSALRTGWYTSVITIELSNIKENKCNGTDAKVKLIKQELDKYKNAVTELQLLMQSTPATNNRARRELPRFMNYTLNNAKKTNVTLSKKRKRRFLGFLLGVGSAIASGVAVCKVLHLEGEVNKIKSALLSTNKAVVSLSNGVSVLTFKVLDLKNYIDKQLLPILNKQSCSISNIETVIEFQQKNNRLLEITREFSVNAGVTTPVSTYMLTNSELLSLINDMPITNDQKKLMSNNVQIVRQQSYSIMCIIKEEVLAYVVQLPLYGVIDTPCWKLHTSPLCTTNTKEGSNICLTRTDRGWYCDNAGSVSFFPQAETCKVQSNRVFCDTMNSLTLPSEVNLCNVDIFNPKYDCKIMTSKTDVSSSVITSLGAIVSCYGKTKCTASNKNRGIIKTFSNGCDYVSNKGVDTVSVGNTLYYVNKQEGKSLYVKGEPIINFYDPLVFPSDEFDASISQVNEKINQSLAFIRKSDELLHNVNAGKSTTNIMITTIIIVIIVILLSLIAVGLLLYCRVRRLLVMINSTHNSPVNAYTLESRMRNPYMGNNSN

SEQ ID NO: 134 - DNA, 1764 bp, Artificial sequence
  recombinant RSV F
atggaactgctgatcctgaaagccaacgctattactactatcctgaccgccgtgacattttgcttcgcatctggacagaacattactgaggaattctaccagtcaacatgcagcgccgtgtccaaaggatacctgagcgccctgcggaccggctggtatacatcagtgattactatcgagctgtccaacatcaaggaaaacaaatgtaatgggaccgacgcaaaggtgaaactgatcaagcaggagctggataagtacaaaaatgccgtgacagaactgcagctgctgatgcagtccacaccagcaactaacaatcgcgcccggagagagctgccccggttcatgaactataccctgaacaatgctaagaaaaccaatgtgacactgtccaagaaacgcaagaggcgcttcctgggatttctgctgggcgtggggtctgccatcgctagtggagtggccgtctgcaaagtcctgcacctggagggcgaagtgaacaagatcaaaagcgccctgctgtccactaacaaggcagtggtcagtctgtcaaatggcgtgtccgtcctgaccttcaaggtgctggacctgaaaaattatattgataagcagctgctgcctatcctgaacaaacagagctgctccatttctaatatcgagacagtgatcgaattccagcagaagaacaatagactgctggagattaccagagagttcagcgtgaacgccggcgtcaccacacccgtgtccacctacatgctgacaaatagtgagctgctgtcactgattaacgacatgcctatcaccaatgatcagaagaaactgatgtccaacaatgtgcagatcgtcagacagcagagttactcaatcatgtgcatcattaaggaggaagtcctggcctacgtggtccagctgccactgtatggcgtgatcgacaccccctgctggaaactgcatacatctcctctgtgcactaccaacacaaaggaaggaagtaatatctgcctgactcgaaccgaccggggatggtactgtgataacgcaggcagcgtgtccttctttccacaggccgagacctgcaaggtccagagcaacagggtgttctgtgacactatgaatagcctgaccctgccttccgaagtcaacctgtgcaatgtggacatctttaatccaaagtacgattgtaagatcatgactagcaagaccgatgtcagctcctctgtgattacttctctgggggccatcgtgagttgctacggaaagacaaaatgtactgccagcaacaaaaatcgcggcatcattaagaccttctccaacgggtgcgactatgtctctaacaagggcgtggatacagtgagtgtcgggaacactctgtactatgtcaataagcaggagggaaaaagcctgtacgtgaagggcgaacccatcattaacttctatgaccccctggtgttcccttccgacgagtttgatgcatctattagtcaggtgaacgaaaaaatcaatcagagtctggcctttattcggaagtcagatgagctgctgcacaacgtgaatgctggcaaatctacaactaacatcatgatcaccacaatcatcatcgtgattatcgtcattctgctgtcactgatcgctgtggggctgctgctgtactgtcgagtgcggagactgctggtcatgattaacagcacccacaattcccccgtcaacgcctacacactggagtctaggatgcgcaatccttatatggggaacaatagcaactgatag

SEQ ID NO: 135 - protein, 588 aa, Artificial sequence
  recombinant RSV F
MELLILKANAITTILTAVTFCFASGQNITEEFYQSTCSAVSKGYLSALRTGWYTSVITIELSNIKENKCNGTDAKVKLIKQELDKYKNAVTELQLLMQSTPATNNRARRELPRFMNYTLNNAKKTNVTLSKKRKRRFLGFLLGVGSAIASGVAVCKVLHLEGEVNKIKSALLSTNKAVVSLSNGVSVLTFKVLDLKNYIDKQLLPILNKQSCSISNIETVIEFQQKNNRLLEITREFSVNAGVTTPVSTYMLTNSELLSLINDMPITNDQKKLMSNNVQIVRQQSYSIMCIIKEEVLAYVVQLPLYGVIDTPCWKLHTSPLCTTNTKEGSNICLTRTDRGWYCDNAGSVSFFPQAETCKVQSNRVFCDTMNSLTLPSEVNLCNVDIFNPKYDCKIMTSKTDVSSSVITSLGAIVSCYGKTKCTASNKNRGIIKTFSNGCDYVSNKGVDTVSVGNTLYYVNKQEGKSLYVKGEPIINFYDPLVFPSDEFDASISQVNEKINQSLAFIRKSDELLHNVNAGKSTTNIMITTQIIMIIIVCILIIIICGILYYLYRVRRLLVMINSTHNSPVNAYTLESRMRNPYMGNNSN

SEQ ID NO: 136 - DNA, 1770 bp, Artificial sequence
  recombinant RSV F
atggaactgctgatcctgaaagccaacgctattactactatcctgaccgccgtgacattttgcttcgcatctggacagaacattactgaggaattctaccagtcaacatgcagcgccgtgtccaaaggatacctgagcgccctgcggaccggctggtatacatcagtgattactatcgagctgtccaacatcaaggaaaacaaatgtaatgggaccgacgcaaaggtgaaactgatcaagcaggagctggataagtacaaaaatgccgtgacagaactgcagctgctgatgcagtccacaccagcaactaacaatcgcgcccggagagagctgccccggttcatgaactataccctgaacaatgctaagaaaaccaatgtgacactgtccaagaaacgcaagaggcgcttcctgggatttctgctgggcgtggggtctgccatcgctagtggagtggccgtctgcaaagtcctgcacctggagggcgaagtgaacaagatcaaaagcgccctgctgtccactaacaaggcagtggtcagtctgtcaaatggcgtgtccgtcctgaccttcaaggtgctggacctgaaaaattatattgataagcagctgctgcctatcctgaacaaacagagctgctccatttctaatatcgagacagtgatcgaattccagcagaagaacaatagactgctggagattaccagagagttcagcgtgaacgccggcgtcaccacacccgtgtccacctacatgctgacaaatagtgagctgctgtcactgattaacgacatgcctatcaccaatgatcagaagaaactgatgtccaacaatgtgcagatcgtcagacagcagagttactcaatcatgtgcatcattaaggaggaagtcctggcctacgtggtccagctgccactgtatggcgtgatcgacaccccctgctggaaactgcatacatctcctctgtgcactaccaacacaaaggaaggaagtaatatctgcctgactcgaaccgaccggggatggtactgtgataacgcaggcagcgtgtccttctttccacaggccgagacctgcaaggtccagagcaacagggtgttctgtgacactatgaatagcctgaccctgccttccgaagtcaacctgtgcaatgtggacatctttaatccaaagtacgattgtaagatcatgactagcaagaccgatgtcagctcctctgtgattacttctctgggggccatcgtgagttgctacggaaagacaaaatgtactgccagcaacaaaaatcgcggcatcattaagaccttctccaacgggtgcgactatgtctctaacaagggcgtggatacagtgagtgtcgggaacactctgtactatgtcaataagcaggagggaaaaagcctgtacgtgaagggcgaacccatcattaacttctatgaccccctggtgttcccttccgacgagtttgatgcatctattagtcaggtgaacgaaaaaatcaatcagagtctggcctttattcggaagtcagatgagctgctgcacaacgtgaatgctggcaaatctacaactaacatcatgatcaccacacagatcattatgatcattatcgtgtgcattctgattatcattatctgtggcatcctgtactatctgtaccgagtgcggagactgctggtcatgattaacagcacccacaattcccccgtcaacgcctacacactggagtctaggatgcgcaatccttatatggggaacaatagcaactgatag

SEQ ID NO: 137 - DNA, 1731 bp, Artificial sequence
  recombinant RSV F
atggaactgctgatcctgaaagccaacgctattactactatcctgaccgccgtgacattttgcttcgcatctggacagaacattactgaggaattctaccagtcaacatgcagcgccgtgtccaaaggatacctgagcgccctgcggaccggctggtatacatcagtgattactatcgagctgtccaacatcaaggaaaacaaatgtaatgggaccgacgcaaaggtgaaactgatcaagcaggagctggataagtacaaaaatgccgtgacagaactgcagctgctgatgcagtccacaccagcaactaacaatcgcgcccggagagagctgccccggttcatgaactataccctgaacaatgctaagaaaaccaatgtgacactgtccaagaaacgcaagaggcgcttcctgggatttctgctgggcgtggggtctgccatcgctagtggagtggccgtctgcaaagtcctgcacctggagggcgaagtgaacaagatcaaaagcgccctgctgtccactaacaaggcagtggtcagtctgtcaaatggcgtgtccgtcctgacctccaaggtgctggacctgaaaaattatattgataagcagctgctgcctatcgtcaacaaacagagctgctccatttctaatatcgagacagtgatcgaattccagcagaagaacaatagactgctggagattaccagagagttcagcgtgaacgccggcgtcaccacacccgtgtccacctacatgctgacaaatagtgagctgctgtcactgattaacgacatgcctatcaccaatgatcagaagaaactgatgtccaacaatgtgcagatcgtcagacagcagagttactcaatcatgtgcatcattaaggaggaagtcctggcctacgtggtccagctgccactgtatggcgtgatcgacaccccctgctggaaactgcatacatctcctctgtgcactaccaacacaaaggaaggaagtaatatctgcctgactcgaaccgaccggggatggtactgtgataacgcaggcagcgtgtccttctttccacaggccgagacctgcaaggtccagagcaacagggtgttctgtgacactatgaatagcctgaccctgccttccgaagtcaacctgtgcaatgtggacatctttaatccaaagtacgattgtaagatcatgactagcaagaccgatgtcagctcctctgtgattacttctctgggggccatcgtgagttgctacggaaagacaaaatgtactgccagcaacaaaaatcgcggcatcattaagaccttctccaacgggtgcgactatgtctctaacaagggcgtggatacagtgagtgtcgggaacactctgtactatgtcaataagcaggagggaaaaagcctgtacgtgaagggcgaacccatcattaacttctatgaccccctggtgttcccttccgacgagtttgatgcatctattagtcaggtgaacgaaaaaatcaatcagagtctggcctttattcggaagtcagatgagctgctgcacaacgtgaatgctggcaaatctacaactaacatcatgatcaccacaatcaccatcattatcgtgatgattatcattctggtcatcattaacatcacaatcattgtggtcatcattaagttccaccggattcagggcaaggaccagaacgataaaaatagcgagccctacatcctgaccaatagacagtga

SEQ ID NO: 138 - DNA, 15 bp, Human parainfluenza virus 1
agggttaaagtaata

SEQ ID NO: 139 - DNA, 21 bp, Human parainfluenza virus 1
taaatacgcgtcccgggaaca

SEQ ID NO: 140 - DNA, 38 bp, Human parainfluenza virus 1
aaagtaagaaaaacttagggtgaatgcgtacgacgcgt

SEQ ID NO: 141 - DNA, 14 bp, Human parainfluenza virus 1
agggtgaatgacaa

SEQ ID NO: 142 - DNA, 21 bp, Human parainfluenza virus 1
cagggcgcgcccccgggaaca

SEQ ID NO: 143 - DNA, 44 bp, Human parainfluenza virus 1
aatcaagtaagaaaaacttagggtgaatggcgtacgggcgcgcc

SEQ ID NO: 144 - DNA, 42 bp, Human parainfluenza virus 1
gcggccgcccgggaagtaagaaaaacttagggtgaatgaaca

SEQ ID NO: 145 - DNA, 31 bp, Human parainfluenza virus 1
cgtacggcggccgcaaaacaattaagaaaaa

SEQ ID NO: 146 - DNA, 15 bp, Human parainfluenza virus 1
acgcgtgccgccacc

SEQ ID NO: 147 - DNA, 37 bp, Human parainfluenza virus 1
aaaagtaagaaaaacttagggtgaatgacgcgtaatg

SEQ ID NO: 148 - DNA, 64 bp, Human parainfluenza virus 3
cttaggattaaagacattgactagaaggtcaagaaaagggaactctataatttcaaaaatgttg

SEQ ID NO: 149 - DNA, 20 bp, Human parainfluenza virus 3
gcttagcgccgccaccatgg

SEQ ID NO: 150 - DNA, 49 bp, Human parainfluenza virus 3
tgatagataataaataagaaaaacttaggattaaagaagcttagcaatg